European Patent Specification EP 3 908 662 B1, published November 20, 2024. Title: ENGINEERED TUBEROUS SCLEROSIS COMPLEX 2 POLYPEPTIDES. Applicant: The Johns Hopkins University. The sequence listing filed with the application follows.

SEQUENCE LISTING (27 sequences)

SEQ ID NO: 1 - protein, 1807 aa, Artificial
  engineered TSC2 polypeptide having an alanine substitution at the serine residue at position S1365 of a human TSC2 polypeptide sequence
MAKPTSKDSGLKEKFKILLGLGTPRPNPRSAEGKQTEFIITAEILRELSMECGLNNRIRMIGQICEVAKTKKFEEHAVEALWKAVADLLQPERPLEARHAVLALLKAIVQGQGERLGVLRALFFKVIKDYPSNEDLHERLEVFKALTDNGRHITYLEEELADFVLQWMDVGLSSEFLLVLVNLVKFNSCYLDEYIARMVQMICLLCVRTASSVDIEVSLQVLDAVVCYNCLPAESLPLFIVTLCRTINVKELCEPCWKLMRNLLGTHLGHSAIYNMCHLMEDRAYMEDAPLLRGAVFFVGMALWGAHRLYSLRNSPTSVLPSFYQAMACPNEVVSYEIVLSITRLIKKYRKELQVVAWDILLNIIERLLQQLQTLDSPELRTIVHDLLTTVEELCDQNEFHGSQERYFELVERCADQRPESSLLNLISYRAQSIHPAKDGWIQNLQALMERFFRSESRGAVRIKVLDVLSFVLLINRQFYEEELINSVVISQLSHIPEDKDHQVRKLATQLLVDLAEGCHTHHFNSLLDIIEKVMARSLSPPPELEERDVAAYSASLEDVKTAVLGLLVILQTKLYTLPASHATRVYEMLVSHIQLHYKHSYTLPIASSIRLQAFDFLLLLRADSLHRLGLPNKDGVVRFSPYCVCDYMEPERGSEKKTSGPLSPPTGPPGPAPAGPAVRLGSVPYSLLFRVLLQCLKQESDWKVLKLVLGRLPESLRYKVLIFTSPCSVDQLCSALCSMLSGPKTLERLRGAPEGFSRTDLHLAVVPVLTALISYHNYLDKTKQREMVYCLEQGLIHRCASQCVVALSICSVEMPDIIIKALPVLVVKLTHISATASMAVPLLEFLSTLARLPHLYRNFAAEQYASVFAISLPYTNPSKFNQYIVCLAHHVIAMWFIRCRLPFRKDFVPFITKGLRSNVLLSFDDTPEKDSFRARSTSLNERPKSLRIARPPKQGLNNSPPVKEFKESSAAEAFRCRSISVSEHVVRSRIQTSLTSASLGSADENSVAQADDSLKNLHLELTETCLDMMARYVFSNFTAVPKRSPVGEFLLAGGRTKTWLVGNKLVTVTTSVGTGTRSLLGLDSGELQSGPESSSSPGVHVRQTKEAPAKLESQAGQQVSRGARDRVRSMSGGHGLRVGALDVPASQFLGSATSPGPRTAPAAKPEKASAGTRVPVQEKTNLAAYVPLLTQGWAEILVRRPTGNTSWLMSLENPLSPFSSDINNMPLQELSNALMAAERFKEHRDTALYKSLSVPAASTAKPPPLPRSNTVASFSSLYQSSCQGQLHRSVSWADSAVVMEEGSPGEVPVLVEPPGLEDVEAALGMDRRTDAYSRSSSVSSQEEKSLHAEELVGRGIPIERVVSAEGGRPSVDLSFQPSQPLSKSSSSPELQTLQDILGDPGDKADVGRLSPEVKARSQSGTLDGESAAWSASGEDSRGQPEGPLPSSSPRSPSGLRPRGYTISDSAPSRRGKRVERDALKSRATASNAEKVPGINPSFVFLQLYHSPFFGDESNKPILLPNESQSFERSVQLLDQIPSYDTHKIAVLYVGEGQSNSELAILSNEHGSYRYTEFLTGLGRLIELKDCQPDKVYLGGLDVCGEDGQFTYCWHDDIMQAVFHIATLMPTKDVDKHRCDKKRHLGNDFVSIVYNDSGEDFKLGTIKGQFNFVHVIVTPLDYECNLVSLQCRKDMEGLVDTSVAKIVSDRNLPFVARQMALHANMASQVHHSRSNPTDIYPSKWIARLRHIKRLRQRICEEAAYSNPSLPLVHPPSHSKAPAQTPAEPTPGYEVGQRKRLISSVEDFTEFV

SEQ ID NO: 2 - protein, 1807 aa, Artificial
  engineered TSC2 polypeptide having a glutamic acid substitution at the serine residue at position S1365 of human TSC2 polypeptide sequence
MAKPTSKDSGLKEKFKILLGLGTPRPNPRSAEGKQTEFIITAEILRELSMECGLNNRIRMIGQICEVAKTKKFEEHAVEALWKAVADLLQPERPLEARHAVLALLKAIVQGQGERLGVLRALFFKVIKDYPSNEDLHERLEVFKALTDNGRHITYLEEELADFVLQWMDVGLSSEFLLVLVNLVKFNSCYLDEYIARMVQMICLLCVRTASSVDIEVSLQVLDAVVCYNCLPAESLPLFIVTLCRTINVKELCEPCWKLMRNLLGTHLGHSAIYNMCHLMEDRAYMEDAPLLRGAVFFVGMALWGAHRLYSLRNSPTSVLPSFYQAMACPNEVVSYEIVLSITRLIKKYRKELQVVAWDILLNIIERLLQQLQTLDSPELRTIVHDLLTTVEELCDQNEFHGSQERYFELVERCADQRPESSLLNLISYRAQSIHPAKDGWIQNLQALMERFFRSESRGAVRIKVLDVLSFVLLINRQFYEEELINSVVISQLSHIPEDKDHQVRKLATQLLVDLAEGCHTHHFNSLLDIIEKVMARSLSPPPELEERDVAAYSASLEDVKTAVLGLLVILQTKLYTLPASHATRVYEMLVSHIQLHYKHSYTLPIASSIRLQAFDFLLLLRADSLHRLGLPNKDGVVRFSPYCVCDYMEPERGSEKKTSGPLSPPTGPPGPAPAGPAVRLGSVPYSLLFRVLLQCLKQESDWKVLKLVLGRLPESLRYKVLIFTSPCSVDQLCSALCSMLSGPKTLERLRGAPEGFSRTDLHLAVVPVLTALISYHNYLDKTKQREMVYCLEQGLIHRCASQCVVALSICSVEMPDIIIKALPVLVVKLTHISATASMAVPLLEFLSTLARLPHLYRNFAAEQYASVFAISLPYTNPSKFNQYIVCLAHHVIAMWFIRCRLPFRKDFVPFITKGLRSNVLLSFDDTPEKDSFRARSTSLNERPKSLRIARPPKQGLNNSPPVKEFKESSAAEAFRCRSISVSEHVVRSRIQTSLTSASLGSADENSVAQADDSLKNLHLELTETCLDMMARYVFSNFTAVPKRSPVGEFLLAGGRTKTWLVGNKLVTVTTSVGTGTRSLLGLDSGELQSGPESSSSPGVHVRQTKEAPAKLESQAGQQVSRGARDRVRSMSGGHGLRVGALDVPASQFLGSATSPGPRTAPAAKPEKASAGTRVPVQEKTNLAAYVPLLTQGWAEILVRRPTGNTSWLMSLENPLSPFSSDINNMPLQELSNALMAAERFKEHRDTALYKSLSVPAASTAKPPPLPRSNTVASFSSLYQSSCQGQLHRSVSWADSAVVMEEGSPGEVPVLVEPPGLEDVEAALGMDRRTDAYSRSSSVSSQEEKSLHAEELVGRGIPIERVVSEEGGRPSVDLSFQPSQPLSKSSSSPELQTLQDILGDPGDKADVGRLSPEVKARSQSGTLDGESAAWSASGEDSRGQPEGPLPSSSPRSPSGLRPRGYTISDSAPSRRGKRVERDALKSRATASNAEKVPGINPSFVFLQLYHSPFFGDESNKPILLPNESQSFERSVQLLDQIPSYDTHKIAVLYVGEGQSNSELAILSNEHGSYRYTEFLTGLGRLIELKDCQPDKVYLGGLDVCGEDGQFTYCWHDDIMQAVFHIATLMPTKDVDKHRCDKKRHLGNDFVSIVYNDSGEDFKLGTIKGQFNFVHVIVTPLDYECNLVSLQCRKDMEGLVDTSVAKIVSDRNLPFVARQMALHANMASQVHHSRSNPTDIYPSKWIARLRHIKRLRQRICEEAAYSNPSLPLVHPPSHSKAPAQTPAEPTPGYEVGQRKRLISSVEDFTEFV

SEQ ID NO: 3 - DNA, 5424 bp, Artificial
  nucleic acid sequence encoding an engineered TSC2 polypeptide having an alanine substitution at the serine residue at position S1365 of a human TSC2 polypeptide sequence
  misc_feature (4095)..(4095): n is a, c, g, or t
atggccaaaccaacaagcaaagattcaggcttgaaggagaagtttaagattctgttgggactgggaacaccgaggccaaatcccaggtctgcagagggtaaacagacggagtttatcatcaccgcggaaatactgagagaactgagcatggaatgtggcctcaacaatcgcatccggatgatagggcagatttgtgaagtcgcaaaaaccaagaaatttgaagagcacgcagtggaagcactctggaaggcggtcgcggatctgttgcagccggagcggccgctggaggcccggcacgcggtgctggctctgctgaaggccatcgtgcaggggcagggcgagcgtttgggggtcctcagagccctcttctttaaggtcatcaaggattacccttccaacgaagaccttcacgaaaggctggaggttttcaaggccctcacagacaatgggagacacatcacctacttggaggaagagctggctgactttgtcctgcagtggatggatgttggcttgtcctcggaattccttctggtgctggtgaacttggtcaaattcaatagctgttacctcgacgagtacatcgcaaggatggttcagatgatctgtctgctgtgcgtccggaccgcgtcctctgtggacatagaggtctccctgcaggtgctggacgccgtggtctgctacaactgcctgccggctgagagcctcccgctgttcatcgttaccctctgtcgcaccatcaacgtcaaggagctctgcgagccttgctggaagctgatgcggaacctccttggcacccacctgggccacagcgccatctacaacatgtgccacctcatggaggacagagcctacatggaggacgcgcccctgctgagaggagccgtgttttttgtgggcatggctctctggggagcccaccggctctattctctcaggaactcgccgacatctgtgttgccatcattttaccaggccatggcatgtccgaacgaggtggtgtcctatgagatcgtcctgtccatcaccaggctcatcaagaagtataggaaggagctccaggtggtggcgtgggacattctgctgaacatcatcgaacggctccttcagcagctccagaccttggacagcccggagctcaggaccatcgtccatgacctgttgaccacggtggaggagctgtgtgaccagaacgagttccacgggtctcaggagagatactttgaactggtggagagatgtgcggaccagaggcctgagtcctccctcctgaacctgatctcctatagagcgcagtccatccacccggccaaggacggctggattcagaacctgcaggcgctgatggagagattcttcaggagcgagtcccgaggcgccgtgcgcatcaaggtgctggacgtgctgtcctttgtgctgctcatcaacaggcagttctatgaggaggagctgattaactcagtggtcatctcgcagctctcccacatccccgaggataaagaccaccaggtccgaaagctggccacccagttgctggtggacctggcagagggctgccacacacaccacttcaacagcctgctggacatcatcgagaaggtgatggcccgctccctctccccacccccggagctggaagaaagggatgtggccgcatactcggcctccttggaggatgtgaagacagccgtcctggggcttctggtcatccttcagaccaagctgtacaccctgcctgcaagccacgccacgcgtgtgtatgagatgctggtcagccacattcagctccactacaagcacagctacaccctgccaatcgcgagcagcatccggctgcaggcctttgacttcctgttgctgctgcgggccgactcactgcaccgcctgggcctgcccaacaaggatggagtcgtgcggttcagcccctactgcgtctgcgactacatggagccagagagaggctctgagaagaagaccagcggccccctttctcctcccacagggcctcctggcccggcgcctgcaggccccgccgtgcggctggggtccgtgccctactccctgctcttccgcgtcctgctgcagtgcttgaagcaggagtctgactggaaggtgctgaagctggttctgggcaggctgcctgagtccctgcgctataaagtgctcatctttacttccccttgcagtgtggaccagctgtgctctgctctctgctccatgctttcaggcccaaagacactggagcggctccgaggcgccccagaaggcttctccagaactgacttgcacctggccgtggttccagtgctgacagcattaatctcttaccataactacctggacaaaaccaaacagcgcgagatggtctactgcctggagcagggcctcatccaccgctgtgccagccagtgcgtcgtggccttgtccatctgcagcgtggagatgcctgacatcatcatcaaggcgctgcctgttctggtggtgaagctcacgcacatctcagccacagccagcatggccgtcccactgctggagttcctgtccactctggccaggctgccgcacctctacaggaactttgccgcggagcagtatgccagtgtgttcgccatctccctgccgtacaccaacccctccaagtttaatcagtacatcgtgtgtctggcccatcacgtcatagccatgtggttcatcaggtgccgcctgcccttccggaaggattttgtccctttcatcactaagggcctgcggtccaatgtcctcttgtcttttgatgacacccccgagaaggacagcttcagggcccggagtactagtctcaacgagagacccaagagtctgaggatagccagaccccccaaacaaggcttgaataactctccacccgtgaaagaattcaaggagagctctgcagccgaggccttccggtgccgcagcatcagtgtgtctgaacatgtggtccgcagcaggatacagacgtccctcaccagtgccagcttggggtctgcagatgagaactccgtggcccaggctgacgatagcctgaaaaacctccacctggagctcacggaaacctgtctggacatgatggctcgatacgtcttctccaacttcacggctgtcccgaagaggtctcctgtgggcgagttcctcctagcgggtggcaggaccaaaacctggctggttgggaacaagcttgtcactgtgacgacaagcgtgggaaccgggacccggtcgttactaggcctggactcgggggagctgcagtccggcccggagtcgagctccagccccggggtgcatgtgagacagaccaaggaggcgccggccaagctggagtcccaggctgggcagcaggtgtcccgtggggcccgggatcgggtccgttccatgtcggggggccatggtcttcgagttggcgccctggacgtgccggcctcccagttcctgggcagtgccacttctccaggaccacggactgcaccagccgcgaaacctgagaaggcctcagctggcacccgggttcctgtgcaggagaagacgaacctggcggcctatgtgcccctgctgacccagggctgggcggagatcctggtccggaggcccacagggaacaccagctggctgatgagcctggagaacccgctcagccctttctcctcggacatcaacaacatgcccctgcaggagctgtctaacgccctcatggcggctgagcgcttcaaggagcaccgggacacagccctgtacaagtcactgtcggtgccggcagccagcacggccaaaccccctcctctgcctcgctccaacacagtggcctctttctcctccctgtaccagtccagctgccaaggacagctgcacaggagcgtttcctgggcagactccgccgtggtcatggaggagggaagtccgggcgaggttcctgtgctggtggagcccccagggttggaggacgttgaggcagcgctaggcatggacaggcgcacggatgcctacagcaggtcgtcctcagtctccagccaggaggagaagtcgctccacgcggaggagctggttggcaggggcatccccatcgagcgagtcgtctcggcngagggtggccggccctctgtggacctctccttccagccctcgcagcccctgagcaagtccagctcctctcccgagctgcagactctgcaggacatcctcggggaccctggggacaaggccgacgtgggccggctgagccctgaggttaaggcccggtcacagtcagggaccctggacggggaaagtgctgcctggtcggcctcgggcgaagacagtcggggccagcccgagggtcccttgccttccagctccccccgctcgcccagtggcctccggccccgaggttacaccatctccgactcggccccatcacgcaggggcaagagagtagagagggacgccttaaagagcagagccacagcctccaatgcagagaaagtgccaggcatcaaccccagtttcgtgttcctgcagctctaccattcccccttctttggcgacgagtcaaacaagccaatcctgctgcccaatgagtcacagtcctttgagcggtcggtgcagctcctcgaccagatcccatcatacgacacccacaagatcgccgtcctgtatgttggagaaggccagagcaacagcgagctcgccatcctgtccaatgagcatggctcctacaggtacacggagttcctgacgggcctgggccggctcatcgagctgaaggactgccagccggacaaggtgtacctgggaggcctggacgtgtgtggtgaggacggccagttcacctactgctggcacgatgacatcatgcaagccgtcttccacatcgccaccctgatgcccaccaaggacgtggacaagcaccgctgcgacaagaagcgccacctgggcaacgactttgtgtccattgtctacaatgactccggtgaggacttcaagcttggcaccatcaagggccagttcaactttgtccacgtgatcgtcaccccgctggactacgagtgcaacctggtgtccctgcagtgcaggaaagacatggagggccttgtggacaccagcgtggccaagatcgtgtctgaccgcaacctgcccttcgtggcccgccagatggccctgcacgcaaatatggcctcacaggtgcatcatagccgctccaaccccaccgatatctacccctccaagtggattgcccggctccgccacatcaagcggctccgccagcggatctgcgaggaagccgcctactccaaccccagcctacctctggtgcaccctccgtcccatagcaaagcccctgcacagactccagccgagcccacacctggctatgaggtgggccagcggaagcgcctcatctcctcggtggaggacttcaccgagtttgtgtga

SEQ ID NO: 4 - DNA, 5424 bp, Artificial
  nucleic acid sequence encoding an engineered TSC2 polypeptide having a glutamic acid substitution at the serine residue at position S1365 of a human TSC2 polypeptide sequence
atggccaaaccaacaagcaaagattcaggcttgaaggagaagtttaagattctgttgggactgggaacaccgaggccaaatcccaggtctgcagagggtaaacagacggagtttatcatcaccgcggaaatactgagagaactgagcatggaatgtggcctcaacaatcgcatccggatgatagggcagatttgtgaagtcgcaaaaaccaagaaatttgaagagcacgcagtggaagcactctggaaggcggtcgcggatctgttgcagccggagcggccgctggaggcccggcacgcggtgctggctctgctgaaggccatcgtgcaggggcagggcgagcgtttgggggtcctcagagccctcttctttaaggtcatcaaggattacccttccaacgaagaccttcacgaaaggctggaggttttcaaggccctcacagacaatgggagacacatcacctacttggaggaagagctggctgactttgtcctgcagtggatggatgttggcttgtcctcggaattccttctggtgctggtgaacttggtcaaattcaatagctgttacctcgacgagtacatcgcaaggatggttcagatgatctgtctgctgtgcgtccggaccgcgtcctctgtggacatagaggtctccctgcaggtgctggacgccgtggtctgctacaactgcctgccggctgagagcctcccgctgttcatcgttaccctctgtcgcaccatcaacgtcaaggagctctgcgagccttgctggaagctgatgcggaacctccttggcacccacctgggccacagcgccatctacaacatgtgccacctcatggaggacagagcctacatggaggacgcgcccctgctgagaggagccgtgttttttgtgggcatggctctctggggagcccaccggctctattctctcaggaactcgccgacatctgtgttgccatcattttaccaggccatggcatgtccgaacgaggtggtgtcctatgagatcgtcctgtccatcaccaggctcatcaagaagtataggaaggagctccaggtggtggcgtgggacattctgctgaacatcatcgaacggctccttcagcagctccagaccttggacagcccggagctcaggaccatcgtccatgacctgttgaccacggtggaggagctgtgtgaccagaacgagttccacgggtctcaggagagatactttgaactggtggagagatgtgcggaccagaggcctgagtcctccctcctgaacctgatctcctatagagcgcagtccatccacccggccaaggacggctggattcagaacctgcaggcgctgatggagagattcttcaggagcgagtcccgaggcgccgtgcgcatcaaggtgctggacgtgctgtcctttgtgctgctcatcaacaggcagttctatgaggaggagctgattaactcagtggtcatctcgcagctctcccacatccccgaggataaagaccaccaggtccgaaagctggccacccagttgctggtggacctggcagagggctgccacacacaccacttcaacagcctgctggacatcatcgagaaggtgatggcccgctccctctccccacccccggagctggaagaaagggatgtggccgcatactcggcctccttggaggatgtgaagacagccgtcctggggcttctggtcatccttcagaccaagctgtacaccctgcctgcaagccacgccacgcgtgtgtatgagatgctggtcagccacattcagctccactacaagcacagctacaccctgccaatcgcgagcagcatccggctgcaggcctttgacttcctgttgctgctgcgggccgactcactgcaccgcctgggcctgcccaacaaggatggagtcgtgcggttcagcccctactgcgtctgcgactacatggagccagagagaggctctgagaagaagaccagcggccccctttctcctcccacagggcctcctggcccggcgcctgcaggccccgccgtgcggctggggtccgtgccctactccctgctcttccgcgtcctgctgcagtgcttgaagcaggagtctgactggaaggtgctgaagctggttctgggcaggctgcctgagtccctgcgctataaagtgctcatctttacttccccttgcagtgtggaccagctgtgctctgctctctgctccatgctttcaggcccaaagacactggagcggctccgaggcgccccagaaggcttctccagaactgacttgcacctggccgtggttccagtgctgacagcattaatctcttaccataactacctggacaaaaccaaacagcgcgagatggtctactgcctggagcagggcctcatccaccgctgtgccagccagtgcgtcgtggccttgtccatctgcagcgtggagatgcctgacatcatcatcaaggcgctgcctgttctggtggtgaagctcacgcacatctcagccacagccagcatggccgtcccactgctggagttcctgtccactctggccaggctgccgcacctctacaggaactttgccgcggagcagtatgccagtgtgttcgccatctccctgccgtacaccaacccctccaagtttaatcagtacatcgtgtgtctggcccatcacgtcatagccatgtggttcatcaggtgccgcctgcccttccggaaggattttgtccctttcatcactaagggcctgcggtccaatgtcctcttgtcttttgatgacacccccgagaaggacagcttcagggcccggagtactagtctcaacgagagacccaagagtctgaggatagccagaccccccaaacaaggcttgaataactctccacccgtgaaagaattcaaggagagctctgcagccgaggccttccggtgccgcagcatcagtgtgtctgaacatgtggtccgcagcaggatacagacgtccctcaccagtgccagcttggggtctgcagatgagaactccgtggcccaggctgacgatagcctgaaaaacctccacctggagctcacggaaacctgtctggacatgatggctcgatacgtcttctccaacttcacggctgtcccgaagaggtctcctgtgggcgagttcctcctagcgggtggcaggaccaaaacctggctggttgggaacaagcttgtcactgtgacgacaagcgtgggaaccgggacccggtcgttactaggcctggactcgggggagctgcagtccggcccggagtcgagctccagccccggggtgcatgtgagacagaccaaggaggcgccggccaagctggagtcccaggctgggcagcaggtgtcccgtggggcccgggatcgggtccgttccatgtcggggggccatggtcttcgagttggcgccctggacgtgccggcctcccagttcctgggcagtgccacttctccaggaccacggactgcaccagccgcgaaacctgagaaggcctcagctggcacccgggttcctgtgcaggagaagacgaacctggcggcctatgtgcccctgctgacccagggctgggcggagatcctggtccggaggcccacagggaacaccagctggctgatgagcctggagaacccgctcagccctttctcctcggacatcaacaacatgcccctgcaggagctgtctaacgccctcatggcggctgagcgcttcaaggagcaccgggacacagccctgtacaagtcactgtcggtgccggcagccagcacggccaaaccccctcctctgcctcgctccaacacagtggcctctttctcctccctgtaccagtccagctgccaaggacagctgcacaggagcgtttcctgggcagactccgccgtggtcatggaggagggaagtccgggcgaggttcctgtgctggtggagcccccagggttggaggacgttgaggcagcgctaggcatggacaggcgcacggatgcctacagcaggtcgtcctcagtctccagccaggaggagaagtcgctccacgcggaggagctggttggcaggggcatccccatcgagcgagtcgtctcggargagggtggccggccctctgtggacctctccttccagccctcgcagcccctgagcaagtccagctcctctcccgagctgcagactctgcaggacatcctcggggaccctggggacaaggccgacgtgggccggctgagccctgaggttaaggcccggtcacagtcagggaccctggacggggaaagtgctgcctggtcggcctcgggcgaagacagtcggggccagcccgagggtcccttgccttccagctccccccgctcgcccagtggcctccggccccgaggttacaccatctccgactcggccccatcacgcaggggcaagagagtagagagggacgccttaaagagcagagccacagcctccaatgcagagaaagtgccaggcatcaaccccagtttcgtgttcctgcagctctaccattcccccttctttggcgacgagtcaaacaagccaatcctgctgcccaatgagtcacagtcctttgagcggtcggtgcagctcctcgaccagatcccatcatacgacacccacaagatcgccgtcctgtatgttggagaaggccagagcaacagcgagctcgccatcctgtccaatgagcatggctcctacaggtacacggagttcctgacgggcctgggccggctcatcgagctgaaggactgccagccggacaaggtgtacctgggaggcctggacgtgtgtggtgaggacggccagttcacctactgctggcacgatgacatcatgcaagccgtcttccacatcgccaccctgatgcccaccaaggacgtggacaagcaccgctgcgacaagaagcgccacctgggcaacgactttgtgtccattgtctacaatgactccggtgaggacttcaagcttggcaccatcaagggccagttcaactttgtccacgtgatcgtcaccccgctggactacgagtgcaacctggtgtccctgcagtgcaggaaagacatggagggccttgtggacaccagcgtggccaagatcgtgtctgaccgcaacctgcccttcgtggcccgccagatggccctgcacgcaaatatggcctcacaggtgcatcatagccgctccaaccccaccgatatctacccctccaagtggattgcccggctccgccacatcaagcggctccgccagcggatctgcgaggaagccgcctactccaaccccagcctacctctggtgcaccctccgtcccatagcaaagcccctgcacagactccagccgagcccacacctggctatgaggtgggccagcggaagcgcctcatctcctcggtggaggacttcaccgagtttgtgtga

SEQ ID NO: 5 - protein, 1807 aa, Homo sapiens
MAKPTSKDSGLKEKFKILLGLGTPRPNPRSAEGKQTEFIITAEILRELSMECGLNNRIRMIGQICEVAKTKKFEEHAVEALWKAVADLLQPERPLEARHAVLALLKAIVQGQGERLGVLRALFFKVIKDYPSNEDLHERLEVFKALTDNGRHITYLEEELADFVLQWMDVGLSSEFLLVLVNLVKFNSCYLDEYIARMVQMICLLCVRTASSVDIEVSLQVLDAVVCYNCLPAESLPLFIVTLCRTINVKELCEPCWKLMRNLLGTHLGHSAIYNMCHLMEDRAYMEDAPLLRGAVFFVGMALWGAHRLYSLRNSPTSVLPSFYQAMACPNEVVSYEIVLSITRLIKKYRKELQVVAWDILLNIIERLLQQLQTLDSPELRTIVHDLLTTVEELCDQNEFHGSQERYFELVERCADQRPESSLLNLISYRAQSIHPAKDGWIQNLQALMERFFRSESRGAVRIKVLDVLSFVLLINRQFYEEELINSVVISQLSHIPEDKDHQVRKLATQLLVDLAEGCHTHHFNSLLDIIEKVMARSLSPPPELEERDVAAYSASLEDVKTAVLGLLVILQTKLYTLPASHATRVYEMLVSHIQLHYKHSYTLPIASSIRLQAFDFLLLLRADSLHRLGLPNKDGVVRFSPYCVCDYMEPERGSEKKTSGPLSPPTGPPGPAPAGPAVRLGSVPYSLLFRVLLQCLKQESDWKVLKLVLGRLPESLRYKVLIFTSPCSVDQLCSALCSMLSGPKTLERLRGAPEGFSRTDLHLAVVPVLTALISYHNYLDKTKQREMVYCLEQGLIHRCASQCVVALSICSVEMPDIIIKALPVLVVKLTHISATASMAVPLLEFLSTLARLPHLYRNFAAEQYASVFAISLPYTNPSKFNQYIVCLAHHVIAMWFIRCRLPFRKDFVPFITKGLRSNVLLSFDDTPEKDSFRARSTSLNERPKSLRIARPPKQGLNNSPPVKEFKESSAAEAFRCRSISVSEHVVRSRIQTSLTSASLGSADENSVAQADDSLKNLHLELTETCLDMMARYVFSNFTAVPKRSPVGEFLLAGGRTKTWLVGNKLVTVTTSVGTGTRSLLGLDSGELQSGPESSSSPGVHVRQTKEAPAKLESQAGQQVSRGARDRVRSMSGGHGLRVGALDVPASQFLGSATSPGPRTAPAAKPEKASAGTRVPVQEKTNLAAYVPLLTQGWAEILVRRPTGNTSWLMSLENPLSPFSSDINNMPLQELSNALMAAERFKEHRDTALYKSLSVPAASTAKPPPLPRSNTVASFSSLYQSSCQGQLHRSVSWADSAVVMEEGSPGEVPVLVEPPGLEDVEAALGMDRRTDAYSRSSSVSSQEEKSLHAEELVGRGIPIERVVSSEGGRPSVDLSFQPSQPLSKSSSSPELQTLQDILGDPGDKADVGRLSPEVKARSQSGTLDGESAAWSASGEDSRGQPEGPLPSSSPRSPSGLRPRGYTISDSAPSRRGKRVERDALKSRATASNAEKVPGINPSFVFLQLYHSPFFGDESNKPILLPNESQSFERSVQLLDQIPSYDTHKIAVLYVGEGQSNSELAILSNEHGSYRYTEFLTGLGRLIELKDCQPDKVYLGGLDVCGEDGQFTYCWHDDIMQAVFHIATLMPTKDVDKHRCDKKRHLGNDFVSIVYNDSGEDFKLGTIKGQFNFVHVIVTPLDYECNLVSLQCRKDMEGLVDTSVAKIVSDRNLPFVARQMALHANMASQVHHSRSNPTDIYPSKWIARLRHIKRLRQRICEEAAYSNPSLPLVHPPSHSKAPAQTPAEPTPGYEVGQRKRLISSVEDFTEFV

SEQ ID NO: 6 - protein, 1814 aa, Mus musculus
MAKPTSKDSGLKEKFKILLGLGTSRPNPRCAEGKQTEFIITSEILRELSGECGLNNRIRMIGQICDVAKTKKLEEHAVEALWKAVSDLLQPERPPEARHAVLTLLKAIVQGQGDRLGVLRALFFKVIKDYPSNEDLHERLEVFKALTDNGRHITYLEEELAEFVLQWMDVGLSSEFLLVLVNLVKFNSCYLDEYIASMVHMICLLCIRTVSSVDIEVSLQVLDAVVCYNCLPAESLPLFIITLCRTINVKELCEPCWKLMRNLLGTHLGHSAIYNMCRIMEDRSYMEDAPLLRGAVFFVGMALWGAHRLYSLKNSPTSVLPSFYEAMTCPNEVVSYEIVLSITRLIKKYRKELQAVTWDILLDIIERLLQQLQNLDSPELKTIVHDLLTTVEELCDQNEFHGSQERYYELVESYADQRPESSLLNLISYRAQSIHPAKDGWIQNLQLLMERFFRNECRSAVAIKVLDVLSFVLLIIRQFYEEELINSVVISQLSHIPEDKDHQVRKLATQLLVDLAEGCHTHHFNSLLDIIEKVMARSLSPPPELEERDLAVHSASLEDVKTAVLGLLVILQTKLYTLPASHATRVYESLISHIQLHYKHGYSLPIASSIRLQAFDFLLLLRADSLHRLGLPNKDGVVRFSPYCLCDCMELDRASEKKASGPLSPPTGPPSPVPMGPAVRLGYLPYSLLFRVLLQCLKQESDWKVLKLVLSRLPESLRYKVLIFTSPCSVDQLSSALCSMLSAPKTLERLRGTPEGFSRTDLHLAVVPVLTALISYHNYLDKTRQREMVYCLEQGLIYRCASQCVVALAICSVEMPDIIIKALPVLVVKLTHISATASMAIPLLEFLSTLARLPHLYRNFVPEQYASVFAISLPYTNPSKFNQYIVCLAHHVIAMWFIRCRLPFRKDFVPYITKGLRSNVLLSFDDTPEKDSFRARSTSLNERPKSLRIARAPKQGLNNSPPVKEFKESCAAEAFRCRSISVSEHVVRSRIQTSLTSASLGSADENSMAQADDNLKNLHLELTETCLDMMARYVFSNFTAVPKRSPVGEFLLAGGRTKTWLVGNKLVTVTTSVGTGTRSLLGLDSGDLQGGSDSSSDPSTHVRQTKEAPAKLESQAGQQVSRGARDRVRSMSGGHGLRVGVLDTSAPYSPGGSASLGPQTAVAAKPEKPPAGAQLPTAEKTNLAAYVPLLTQGWAEILVRRPTGNTSWLMSLENPLSPFSSDINNMPLQELSNALMAAERFKEHGHAPVQVIVSATGCTAKPPTLPRSNTVASFSSLYQPSCQGQLHRSVSWADSAMVLEEGSPGETQVPVEPPELEDFEAALGTDRHCQRPDTYSRSSSASSQEEKSHLEELAAGGIPIERAISSEGARPAVDLSFQPSQPLSKSSSSPELQTLQDILGDLGDKIDIGRLSPEAKVRSQSGILDGEAATWSATGEESRITVPPEGPLPSSSPRSPSGLRPRGYTISDSAPSRRGKRVERDNFKSRAAASSAEKVPGINPSFVFLQLYHSPFFGDESNKPILLPNESFERSVQLLDQIPSYDTHKIAVLYVGEGQSSSELAILSNEHGSYRYTEFLTGLGRLIELKDCQPDKVYLGGLDVCGEDGQFTYCWHDDIMQAVFHIATLMPTKDVDKHRCDKKRHLGNDFVSIIYNDSGEDFKLGTIKQGQFNFVHVIITPLDYKCNLLTLQCRKDGPACKCEWWRQPGEIVVWALPVVMELTVTILLCHLQMASQVHHSRSNPTDIYPSKWIARLRHIKRLRQRIREEVHYSNPSLPLMHPPAHTKAPAQAPEATPTYETGQRKRLISSVDDFTEFV

SEQ ID NO: 7 - protein, 1809 aa, Rattus rattus
MAKPTSKDSGLKEKFKILLGLGTSRPNPRCAEGKQTEFIITAEILRELSGECGLNNRIRMIGQICDVAKTKKLEEHAVEALWKAVSDLLQPERPPEARHAVLALLKAIVQGQGDRLGVLRALFFKVIKDYPSNEDLHERLEVFKALTDNGRHITYLEEELAEFVLQWMDVGLSSEFLLVLVNLVKFNSCYLDEYIAPMVHMICLLCIRTVSSVDIEVSLQVLDAVVCYNCLPAESLPLFIITLCRTVNVKELCEPCWKLMRNLLGTHLGHSAIYNMCRIMENRSYMEDAPLLRGAVFFVGMALWGAHRLYSLKNSPTSVLPSFYEAMTCPNEVVSYEIVLSITRLIKKYRKELQAVTWDILLDIIERLLQQLQNLDSPELRTIVHDLLTTVEELCDQNEFHGSQERYYELVESYADQRPESSLLNLITYRAQSIHPAKDGWIQNLQLLMERFFRNECRSAVRIKVLDVLSFVLLINRQFYEEELINSVVISQLSHIPEDKDHQVRKLATQLLVDLAEGCHTHHFNSLLDIIEKVMARSLSPPLELEERDLAVYSASLEDVKTAVLGLLVILQTKLYTLPASHATRVYETLISHIQLHYKHGYSLPIASSIRLQAFDFLLLLRADSLHRLGLPNKDGVVRFSPYCLCDCAELDRASEKKASGPLSPPTGPPSPVPTGPAVRLGHLPYSLLFRVLLQCLKQETDWKVLKLVLSKLPESLRYKVLIFTSPCSVDQLSSALCSMLSAPKTLERLRGTPEGFSRTDLHLAVVPVLTALISYHNYLDKTRQREMVYCLEQGLIYRCASQCVVALAICSVEMPDIIIKALPVLVVKLTHISATASMAIPLLEFLSTLARLPHLYRNFAAEQYASVFAISLPYTNPSKFNQYIVCLAHHVIAMWFIRCRLPFRKDFVPYITKGLRSNVLLSFDDTPEKDKFRARSTSLNERPKSLRIARAPKQGLNNSPPVKEFKESCAAEAFRCRSISVSEHVVRSRIQTSLTSASLGSADENSMAQADDNLKNLHLELTETCLDMMARYVFSNFTAVPKRSPVGEFLLAGGRTKTWLVGNKLVTVTTSVGTGTRSLLGLDSGDLQGGSASSSDPGTHVRQTKEAPAKLESQAGQQVSRGARDRVRSMSGGHGLRVGVLDTSAPYTPGGPASLGAQAAPAARPEKPCAGAQLPAAEKANLAAYVPLLTQGWAEILVRRPTGNTSWLMSLENPLSPFSSDINNMPLQELSNALMAAERFKEHRDTALYKSLSVPAAGTAKPPTLPRSNTVASFSSLYQPSCQGQLHRSVSWADSAVVLEEGSPGEAHVPVEPPELEDFEAALGTDRHCQRPDAYSRSSSASSQEEKSHLEELAAGGIPIERAISSEGARPTVDLSFQPSQPLSKSSSSPELQTLQDILGDLGDKTDIGRLSPEAKVRSQSGILDGEAATWSAPGEESRITVPPEGPLPSSSPRSPSGLRPRGYTISDSAPSRRGKRVERDNFKSRTAASSAEKVPGINPSFVFLQLYHSPFCGDESNKPILLPNESFERSVQLLDQIPSYDTHKIAVLYVGEGQSSSELAILSNEHGSYRYTEFLTGLGRLIELKDCQPDKVYLGGLDVCGEDGQFTYCWHDDIMQAVFHIATLMPTKDVDKHRCDKKRHLGNDFVSIIYNDSGEDFKLGTIKGQFNFVHVIITPLDYKCNLLTLQCRKDMEGLVDTSVAKIVSDRNLSFVARQMALHANMASQVHHRRSNPTDIYPSKWIARLRHIKRLRQRIREEVHYSNPSLPLMHPPAHTKVPAQAPTEATPTYETGQRKRLISSVDDFTEFV

SEQ ID NO: 8 - protein, 1814 aa, Artificial
  engineered TSC2 polypeptide having an alanine substitution at the serine residue at position S1366 of a mouse TSC2 polypeptide sequence
MAKPTSKDSGLKEKFKILLGLGTSRPNPRCAEGKQTEFIITSEILRELSGECGLNNRIRMIGQICDVAKTKKLEEHAVEALWKAVSDLLQPERPPEARHAVLTLLKAIVQGQGDRLGVLRALFFKVIKDYPSNEDLHERLEVFKALTDNGRHITYLEEELAEFVLQWMDVGLSSEFLLVLVNLVKFNSCYLDEYIASMVHMICLLCIRTVSSVDIEVSLQVLDAVVCYNCLPAESLPLFIITLCRTINVKELCEPCWKLMRNLLGTHLGHSAIYNMCRIMEDRSYMEDAPLLRGAVFFVGMALWGAHRLYSLKNSPTSVLPSFYEAMTCPNEVVSYEIVLSITRLIKKYRKELQAVTWDILLDIIERLLQQLQNLDSPELKTIVHDLLTTVEELCDQNEFHGSQERYYELVESYADQRPESSLLNLISYRAQSIHPAKDGWIQNLQLLMERFFRNECRSAVAIKVLDVLSFVLLIIRQFYEEELINSVVISQLSHIPEDKDHQVRKLATQLLVDLAEGCHTHHFNSLLDIIEKVMARSLSPPPELEERDLAVHSASLEDVKTAVLGLLVILQTKLYTLPASHATRVYESLISHIQLHYKHGYSLPIASSIRLQAFDFLLLLRADSLHRLGLPNKDGVVRFSPYCLCDCMELDRASEKKASGPLSPPTGPPSPVPMGPAVRLGYLPYSLLFRVLLQCLKQESDWKVLKLVLSRLPESLRYKVLIFTSPCSVDQLSSALCSMLSAPKTLERLRGTPEGFSRTDLHLAVVPVLTALISYHNYLDKTRQREMVYCLEQGLIYRCASQCVVALAICSVEMPDIIIKALPVLVVKLTHISATASMAIPLLEFLSTLARLPHLYRNFVPEQYASVFAISLPYTNPSKFNQYIVCLAHHVIAMWFIRCRLPFRKDFVPYITKGLRSNVLLSFDDTPEKDSFRARSTSLNERPKSLRIARAPKQGLNNSPPVKEFKESCAAEAFRCRSISVSEHVVRSRIQTSLTSASLGSADENSMAQADDNLKNLHLELTETCLDMMARYVFSNFTAVPKRSPVGEFLLAGGRTKTWLVGNKLVTVTTSVGTGTRSLLGLDSGDLQGGSDSSSDPSTHVRQTKEAPAKLESQAGQQVSRGARDRVRSMSGGHGLRVGVLDTSAPYSPGGSASLGPQTAVAAKPEKPPAGAQLPTAEKTNLAAYVPLLTQGWAEILVRRPTGNTSWLMSLENPLSPFSSDINNMPLQELSNALMAAERFKEHGHAPVQVIVSATGCTAKPPTLPRSNTVASFSSLYQPSCQGQLHRSVSWADSAMVLEEGSPGETQVPVEPPELEDFEAALGTDRHCQRPDTYSRSSSASSQEEKSHLEELAAGGIPIERAISAEGARPAVDLSFQPSQPLSKSSSSPELQTLQDILGDLGDKIDIGRLSPEAKVRSQSGILDGEAATWSATGEESRITVPPEGPLPSSSPRSPSGLRPRGYTISDSAPSRRGKRVERDNFKSRAAASSAEKVPGINPSFVFLQLYHSPFFGDESNKPILLPNESFERSVQLLDQIPSYDTHKIAVLYVGEGQSSSELAILSNEHGSYRYTEFLTGLGRLIELKDCQPDKVYLGGLDVCGEDGQFTYCWHDDIMQAVFHIATLMPTKDVDKHRCDKKRHLGNDFVSIIYNDSGEDFKLGTIKQGQFNFVHVIITPLDYKCNLLTLQCRKDGPACKCEWWRQPGEIVVWALPVVMELTVTILLCHLQMASQVHHSRSNPTDIYPSKWIARLRHIKRLRQRIREEVHYSNPSLPLMHPPAHTKAPAQAPEATPTYETGQRKRLISSVDDFTEFV

SEQ ID NO: 9 - protein, 1809 aa, Artificial
  engineered TSC2 polypeptide having an alanine substitution at the serine residue at position S1367 of rat TSC2 polypeptide sequence
MAKPTSKDSGLKEKFKILLGLGTSRPNPRCAEGKQTEFIITAEILRELSGECGLNNRIRMIGQICDVAKTKKLEEHAVEALWKAVSDLLQPERPPEARHAVLALLKAIVQGQGDRLGVLRALFFKVIKDYPSNEDLHERLEVFKALTDNGRHITYLEEELAEFVLQWMDVGLSSEFLLVLVNLVKFNSCYLDEYIAPMVHMICLLCIRTVSSVDIEVSLQVLDAVVCYNCLPAESLPLFIITLCRTVNVKELCEPCWKLMRNLLGTHLGHSAIYNMCRIMENRSYMEDAPLLRGAVFFVGMALWGAHRLYSLKNSPTSVLPSFYEAMTCPNEVVSYEIVLSITRLIKKYRKELQAVTWDILLDIIERLLQQLQNLDSPELRTIVHDLLTTVEELCDQNEFHGSQERYYELVESYADQRPESSLLNLITYRAQSIHPAKDGWIQNLQLLMERFFRNECRSAVRIKVLDVLSFVLLINRQFYEEELINSVVISQLSHIPEDKDHQVRKLATQLLVDLAEGCHTHHFNSLLDIIEKVMARSLSPPLELEERDLAVYSASLEDVKTAVLGLLVILQTKLYTLPASHATRVYETLISHIQLHYKHGYSLPIASSIRLQAFDFLLLLRADSLHRLGLPNKDGVVRFSPYCLCDCAELDRASEKKASGPLSPPTGPPSPVPTGPAVRLGHLPYSLLFRVLLQCLKQETDWKVLKLVLSKLPESLRYKVLIFTSPCSVDQLSSALCSMLSAPKTLERLRGTPEGFSRTDLHLAVVPVLTALISYHNYLDKTRQREMVYCLEQGLIYRCASQCVVALAICSVEMPDIIIKALPVLVVKLTHISATASMAIPLLEFLSTLARLPHLYRNFAAEQYASVFAISLPYTNPSKFNQYIVCLAHHVIAMWFIRCRLPFRKDFVPYITKGLRSNVLLSFDDTPEKDKFRARSTSLNERPKSLRIARAPKQGLNNSPPVKEFKESCAAEAFRCRSISVSEHVVRSRIQTSLTSASLGSADENSMAQADDNLKNLHLELTETCLDMMARYVFSNFTAVPKRSPVGEFLLAGGRTKTWLVGNKLVTVTTSVGTGTRSLLGLDSGDLQGGSASSSDPGTHVRQTKEAPAKLESQAGQQVSRGARDRVRSMSGGHGLRVGVLDTSAPYTPGGPASLGAQAAPAARPEKPCAGAQLPAAEKANLAAYVPLLTQGWAEILVRRPTGNTSWLMSLENPLSPFSSDINNMPLQELSNALMAAERFKEHRDTALYKSLSVPAAGTAKPPTLPRSNTVASFSSLYQPSCQGQLHRSVSWADSAVVLEEGSPGEAHVPVEPPELEDFEAALGTDRHCQRPDAYSRSSSASSQEEKSHLEELAAGGIPIERAISAEGARPTVDLSFQPSQPLSKSSSSPELQTLQDILGDLGDKTDIGRLSPEAKVRSQSGILDGEAATWSAPGEESRITVPPEGPLPSSSPRSPSGLRPRGYTISDSAPSRRGKRVERDNFKSRTAASSAEKVPGINPSFVFLQLYHSPFCGDESNKPILLPNESFERSVQLLDQIPSYDTHKIAVLYVGEGQSSSELAILSNEHGSYRYTEFLTGLGRLIELKDCQPDKVYLGGLDVCGEDGQFTYCWHDDIMQAVFHIATLMPTKDVDKHRCDKKRHLGNDFVSIIYNDSGEDFKLGTIKGQFNFVHVIITPLDYKCNLLTLQCRKDMEGLVDTSVAKIVSDRNLSFVARQMALHANMASQVHHRRSNPTDIYPSKWIARLRHIKRLRQRIREEVHYSNPSLPLMHPPAHTKVPAQAPTEATPTYETGQRKRLISSVDDFTEFV

SEQ ID NO: 10 - protein, 1814 aa, Artificial
  engineered TSC2 polypeptide having a glutamic acid substitution at the serine residue at position S1366 of a mouse TSC2 polypeptide sequence
MAKPTSKDSGLKEKFKILLGLGTSRPNPRCAEGKQTEFIITSEILRELSGECGLNNRIRMIGQICDVAKTKKLEEHAVEALWKAVSDLLQPERPPEARHAVLTLLKAIVQGQGDRLGVLRALFFKVIKDYPSNEDLHERLEVFKALTDNGRHITYLEEELAEFVLQWMDVGLSSEFLLVLVNLVKFNSCYLDEYIASMVHMICLLCIRTVSSVDIEVSLQVLDAVVCYNCLPAESLPLFIITLCRTINVKELCEPCWKLMRNLLGTHLGHSAIYNMCRIMEDRSYMEDAPLLRGAVFFVGMALWGAHRLYSLKNSPTSVLPSFYEAMTCPNEVVSYEIVLSITRLIKKYRKELQAVTWDILLDIIERLLQQLQNLDSPELKTIVHDLLTTVEELCDQNEFHGSQERYYELVESYADQRPESSLLNLISYRAQSIHPAKDGWIQNLQLLMERFFRNECRSAVAIKVLDVLSFVLLIIRQFYEEELINSVVISQLSHIPEDKDHQVRKLATQLLVDLAEGCHTHHFNSLLDIIEKVMARSLSPPPELEERDLAVHSASLEDVKTAVLGLLVILQTKLYTLPASHATRVYESLISHIQLHYKHGYSLPIASSIRLQAFDFLLLLRADSLHRLGLPNKDGVVRFSPYCLCDCMELDRASEKKASGPLSPPTGPPSPVPMGPAVRLGYLPYSLLFRVLLQCLKQESDWKVLKLVLSRLPESLRYKVLIFTSPCSVDQLSSALCSMLSAPKTLERLRGTPEGFSRTDLHLAVVPVLTALISYHNYLDKTRQREMVYCLEQGLIYRCASQCVVALAICSVEMPDIIIKALPVLVVKLTHISATASMAIPLLEFLSTLARLPHLYRNFVPEQYASVFAISLPYTNPSKFNQYIVCLAHHVIAMWFIRCRLPFRKDFVPYITKGLRSNVLLSFDDTPEKDSFRARSTSLNERPKSLRIARAPKQGLNNSPPVKEFKESCAAEAFRCRSISVSEHVVRSRIQTSLTSASLGSADENSMAQADDNLKNLHLELTETCLDMMARYVFSNFTAVPKRSPVGEFLLAGGRTKTWLVGNKLVTVTTSVGTGTRSLLGLDSGDLQGGSDSSSDPSTHVRQTKEAPAKLESQAGQQVSRGARDRVRSMSGGHGLRVGVLDTSAPYSPGGSASLGPQTAVAAKPEKPPAGAQLPTAEKTNLAAYVPLLTQGWAEILVRRPTGNTSWLMSLENPLSPFSSDINNMPLQELSNALMAAERFKEHGHAPVQVIVSATGCTAKPPTLPRSNTVASFSSLYQPSCQGQLHRSVSWADSAMVLEEGSPGETQVPVEPPELEDFEAALGTDRHCQRPDTYSRSSSASSQEEKSHLEELAAGGIPIERAISEEGARPAVDLSFQPSQPLSKSSSSPELQTLQDILGDLGDKIDIGRLSPEAKVRSQSGILDGEAATWSATGEESRITVPPEGPLPSSSPRSPSGLRPRGYTISDSAPSRRGKRVERDNFKSRAAASSAEKVPGINPSFVFLQLYHSPFFGDESNKPILLPNESFERSVQLLDQIPSYDTHKIAVLYVGEGQSSSELAILSNEHGSYRYTEFLTGLGRLIELKDCQPDKVYLGGLDVCGEDGQFTYCWHDDIMQAVFHIATLMPTKDVDKHRCDKKRHLGNDFVSIIYNDSGEDFKLGTIKQGQFNFVHVIITPLDYKCNLLTLQCRKDGPACKCEWWRQPGEIVVWALPVVMELTVTILLCHLQMASQVHHSRSNPTDIYPSKWIARLRHIKRLRQRIREEVHYSNPSLPLMHPPAHTKAPAQAPEATPTYETGQRKRLISSVDDFTEFV

SEQ ID NO: 11 - protein, 1809 aa, Artificial
  engineered TSC2 polypeptide having a glutamic acid substitution at the serine residue at position S1367 of a rat TSC2 polypeptide sequence
MAKPTSKDSGLKEKFKILLGLGTSRPNPRCAEGKQTEFIITAEILRELSGECGLNNRIRMIGQICDVAKTKKLEEHAVEALWKAVSDLLQPERPPEARHAVLALLKAIVQGQGDRLGVLRALFFKVIKDYPSNEDLHERLEVFKALTDNGRHITYLEEELAEFVLQWMDVGLSSEFLLVLVNLVKFNSCYLDEYIAPMVHMICLLCIRTVSSVDIEVSLQVLDAVVCYNCLPAESLPLFIITLCRTVNVKELCEPCWKLMRNLLGTHLGHSAIYNMCRIMENRSYMEDAPLLRGAVFFVGMALWGAHRLYSLKNSPTSVLPSFYEAMTCPNEVVSYEIVLSITRLIKKYRKELQAVTWDILLDIIERLLQQLQNLDSPELRTIVHDLLTTVEELCDQNEFHGSQERYYELVESYADQRPESSLLNLITYRAQSIHPAKDGWIQNLQLLMERFFRNECRSAVRIKVLDVLSFVLLINRQFYEEELINSVVISQLSHIPEDKDHQVRKLATQLLVDLAEGCHTHHFNSLLDIIEKVMARSLSPPLELEERDLAVYSASLEDVKTAVLGLLVILQTKLYTLPASHATRVYETLISHIQLHYKHGYSLPIASSIRLQAFDFLLLLRADSLHRLGLPNKDGVVRFSPYCLCDCAELDRASEKKASGPLSPPTGPPSPVPTGPAVRLGHLPYSLLFRVLLQCLKQETDWKVLKLVLSKLPESLRYKVLIFTSPCSVDQLSSALCSMLSAPKTLERLRGTPEGFSRTDLHLAVVPVLTALISYHNYLDKTRQREMVYCLEQGLIYRCASQCVVALAICSVEMPDIIIKALPVLVVKLTHISATASMAIPLLEFLSTLARLPHLYRNFAAEQYASVFAISLPYTNPSKFNQYIVCLAHHVIAMWFIRCRLPFRKDFVPYITKGLRSNVLLSFDDTPEKDKFRARSTSLNERPKSLRIARAPKQGLNNSPPVKEFKESCAAEAFRCRSISVSEHVVRSRIQTSLTSASLGSADENSMAQADDNLKNLHLELTETCLDMMARYVFSNFTAVPKRSPVGEFLLAGGRTKTWLVGNKLVTVTTSVGTGTRSLLGLDSGDLQGGSASSSDPGTHVRQTKEAPAKLESQAGQQVSRGARDRVRSMSGGHGLRVGVLDTSAPYTPGGPASLGAQAAPAARPEKPCAGAQLPAAEKANLAAYVPLLTQGWAEILVRRPTGNTSWLMSLENPLSPFSSDINNMPLQELSNALMAAERFKEHRDTALYKSLSVPAAGTAKPPTLPRSNTVASFSSLYQPSCQGQLHRSVSWADSAVVLEEGSPGEAHVPVEPPELEDFEAALGTDRHCQRPDAYSRSSSASSQEEKSHLEELAAGGIPIERAISEEGARPTVDLSFQPSQPLSKSSSSPELQTLQDILGDLGDKTDIGRLSPEAKVRSQSGILDGEAATWSAPGEESRITVPPEGPLPSSSPRSPSGLRPRGYTISDSAPSRRGKRVERDNFKSRTAASSAEKVPGINPSFVFLQLYHSPFCGDESNKPILLPNESFERSVQLLDQIPSYDTHKIAVLYVGEGQSSSELAILSNEHGSYRYTEFLTGLGRLIELKDCQPDKVYLGGLDVCGEDGQFTYCWHDDIMQAVFHIATLMPTKDVDKHRCDKKRHLGNDFVSIIYNDSGEDFKLGTIKGQFNFVHVIITPLDYKCNLLTLQCRKDMEGLVDTSVAKIVSDRNLSFVARQMALHANMASQVHHRRSNPTDIYPSKWIARLRHIKRLRQRIREEVHYSNPSLPLMHPPAHTKVPAQAPTEATPTYETGQRKRLISSVDDFTEFV

SEQ ID NO: 12 - protein, 1807 aa, Artificial
  engineered TSC2 polypeptide having an alanine substitution at the serine residue at position S1364 of a human TSC2 polypeptide sequence
MAKPTSKDSGLKEKFKILLGLGTPRPNPRSAEGKQTEFIITAEILRELSMECGLNNRIRMIGQICEVAKTKKFEEHAVEALWKAVADLLQPERPLEARHAVLALLKAIVQGQGERLGVLRALFFKVIKDYPSNEDLHERLEVFKALTDNGRHITYLEEELADFVLQWMDVGLSSEFLLVLVNLVKFNSCYLDEYIARMVQMICLLCVRTASSVDIEVSLQVLDAVVCYNCLPAESLPLFIVTLCRTINVKELCEPCWKLMRNLLGTHLGHSAIYNMCHLMEDRAYMEDAPLLRGAVFFVGMALWGAHRLYSLRNSPTSVLPSFYQAMACPNEVVSYEIVLSITRLIKKYRKELQVVAWDILLNIIERLLQQLQTLDSPELRTIVHDLLTTVEELCDQNEFHGSQERYFELVERCADQRPESSLLNLISYRAQSIHPAKDGWIQNLQALMERFFRSESRGAVRIKVLDVLSFVLLINRQFYEEELINSVVISQLSHIPEDKDHQVRKLATQLLVDLAEGCHTHHFNSLLDIIEKVMARSLSPPPELEERDVAAYSASLEDVKTAVLGLLVILQTKLYTLPASHATRVYEMLVSHIQLHYKHSYTLPIASSIRLQAFDFLLLLRADSLHRLGLPNKDGVVRFSPYCVCDYMEPERGSEKKTSGPLSPPTGPPGPAPAGPAVRLGSVPYSLLFRVLLQCLKQESDWKVLKLVLGRLPESLRYKVLIFTSPCSVDQLCSALCSMLSGPKTLERLRGAPEGFSRTDLHLAVVPVLTALISYHNYLDKTKQREMVYCLEQGLIHRCASQCVVALSICSVEMPDIIIKALPVLVVKLTHISATASMAVPLLEFLSTLARLPHLYRNFAAEQYASVFAISLPYTNPSKFNQYIVCLAHHVIAMWFIRCRLPFRKDFVPFITKGLRSNVLLSFDDTPEKDSFRARSTSLNERPKSLRIARPPKQGLNNSPPVKEFKESSAAEAFRCRSISVSEHVVRSRIQTSLTSASLGSADENSVAQADDSLKNLHLELTETCLDMMARYVFSNFTAVPKRSPVGEFLLAGGRTKTWLVGNKLVTVTTSVGTGTRSLLGLDSGELQSGPESSSSPGVHVRQTKEAPAKLESQAGQQVSRGARDRVRSMSGGHGLRVGALDVPASQFLGSATSPGPRTAPAAKPEKASAGTRVPVQEKTNLAAYVPLLTQGWAEILVRRPTGNTSWLMSLENPLSPFSSDINNMPLQELSNALMAAERFKEHRDTALYKSLSVPAASTAKPPPLPRSNTVASFSSLYQSSCQGQLHRSVSWADSAVVMEEGSPGEVPVLVEPPGLEDVEAALGMDRRTDAYSRSSSVSSQEEKSLHAEELVGRGIPIERVVASEGGRPSVDLSFQPSQPLSKSSSSPELQTLQDILGDPGDKADVGRLSPEVKARSQSGTLDGESAAWSASGEDSRGQPEGPLPSSSPRSPSGLRPRGYTISDSAPSRRGKRVERDALKSRATASNAEKVPGINPSFVFLQLYHSPFFGDESNKPILLPNESQSFERSVQLLDQIPSYDTHKIAVLYVGEGQSNSELAILSNEHGSYRYTEFLTGLGRLIELKDCQPDKVYLGGLDVCGEDGQFTYCWHDDIMQAVFHIATLMPTKDVDKHRCDKKRHLGNDFVSIVYNDSGEDFKLGTIKGQFNFVHVIVTPLDYECNLVSLQCRKDMEGLVDTSVAKIVSDRNLPFVARQMALHANMASQVHHSRSNPTDIYPSKWIARLRHIKRLRQRICEEAAYSNPSLPLVHPPSHSKAPAQTPAEPTPGYEVGQRKRLISSVEDFTEFV

SEQ ID NO: 13 - protein, 1807 aa, Artificial
  engineered TSC2 polypeptide having a glutamic acid substitution at the serine residue at position S1364 of a human TSC2 polypeptide sequence
MAKPTSKDSGLKEKFKILLGLGTPRPNPRSAEGKQTEFIITAEILRELSMECGLNNRIRMIGQICEVAKTKKFEEHAVEALWKAVADLLQPERPLEARHAVLALLKAIVQGQGERLGVLRALFFKVIKDYPSNEDLHERLEVFKALTDNGRHITYLEEELADFVLQWMDVGLSSEFLLVLVNLVKFNSCYLDEYIARMVQMICLLCVRTASSVDIEVSLQVLDAVVCYNCLPAESLPLFIVTLCRTINVKELCEPCWKLMRNLLGTHLGHSAIYNMCHLMEDRAYMEDAPLLRGAVFFVGMALWGAHRLYSLRNSPTSVLPSFYQAMACPNEVVSYEIVLSITRLIKKYRKELQVVAWDILLNIIERLLQQLQTLDSPELRTIVHDLLTTVEELCDQNEFHGSQERYFELVERCADQRPESSLLNLISYRAQSIHPAKDGWIQNLQALMERFFRSESRGAVRIKVLDVLSFVLLINRQFYEEELINSVVISQLSHIPEDKDHQVRKLATQLLVDLAEGCHTHHFNSLLDIIEKVMARSLSPPPELEERDVAAYSASLEDVKTAVLGLLVILQTKLYTLPASHATRVYEMLVSHIQLHYKHSYTLPIASSIRLQAFDFLLLLRADSLHRLGLPNKDGVVRFSPYCVCDYMEPERGSEKKTSGPLSPPTGPPGPAPAGPAVRLGSVPYSLLFRVLLQCLKQESDWKVLKLVLGRLPESLRYKVLIFTSPCSVDQLCSALCSMLSGPKTLERLRGAPEGFSRTDLHLAVVPVLTALISYHNYLDKTKQREMVYCLEQGLIHRCASQCVVALSICSVEMPDIIIKALPVLVVKLTHISATASMAVPLLEFLSTLARLPHLYRNFAAEQYASVFAISLPYTNPSKFNQYIVCLAHHVIAMWFIRCRLPFRKDFVPFITKGLRSNVLLSFDDTPEKDSFRARSTSLNERPKSLRIARPPKQGLNNSPPVKEFKESSAAEAFRCRSISVSEHVVRSRIQTSLTSASLGSADENSVAQADDSLKNLHLELTETCLDMMARYVFSNFTAVPKRSPVGEFLLAGGRTKTWLVGNKLVTVTTSVGTGTRSLLGLDSGELQSGPESSSSPGVHVRQTKEAPAKLESQAGQQVSRGARDRVRSMSGGHGLRVGALDVPASQFLGSATSPGPRTAPAAKPEKASAGTRVPVQEKTNLAAYVPLLTQGWAEILVRRPTGNTSWLMSLENPLSPFSSDINNMPLQELSNALMAAERFKEHRDTALYKSLSVPAASTAKPPPLPRSNTVASFSSLYQSSCQGQLHRSVSWADSAVVMEEGSPGEVPVLVEPPGLEDVEAALGMDRRTDAYSRSSSVSSQEEKSLHAEELVGRGIPIERVVESEGGRPSVDLSFQPSQPLSKSSSSPELQTLQDILGDPGDKADVGRLSPEVKARSQSGTLDGESAAWSASGEDSRGQPEGPLPSSSPRSPSGLRPRGYTISDSAPSRRGKRVERDALKSRATASNAEKVPGINPSFVFLQLYHSPFFGDESNKPILLPNESQSFERSVQLLDQIPSYDTHKIAVLYVGEGQSNSELAILSNEHGSYRYTEFLTGLGRLIELKDCQPDKVYLGGLDVCGEDGQFTYCWHDDIMQAVFHIATLMPTKDVDKHRCDKKRHLGNDFVSIVYNDSGEDFKLGTIKGQFNFVHVIVTPLDYECNLVSLQCRKDMEGLVDTSVAKIVSDRNLPFVARQMALHANMASQVHHSRSNPTDIYPSKWIARLRHIKRLRQRICEEAAYSNPSLPLVHPPSHSKAPAQTPAEPTPGYEVGQRKRLISSVEDFTEFV

SEQ ID NO: 14 - DNA, 5424 bp, Artificial
  nucleic acid sequence encoding an amino acid sequence of an exemplary engineered TSC2 polypeptide having an alanine substitution at the serine residue at position S1364 of a human TSC2 polypeptide sequence
  misc_feature (4092)..(4092): n is a, c, g, or t
atggccaaaccaacaagcaaagattcaggcttgaaggagaagtttaagattctgttgggactgggaacaccgaggccaaatcccaggtctgcagagggtaaacagacggagtttatcatcaccgcggaaatactgagagaactgagcatggaatgtggcctcaacaatcgcatccggatgatagggcagatttgtgaagtcgcaaaaaccaagaaatttgaagagcacgcagtggaagcactctggaaggcggtcgcggatctgttgcagccggagcggccgctggaggcccggcacgcggtgctggctctgctgaaggccatcgtgcaggggcagggcgagcgtttgggggtcctcagagccctcttctttaaggtcatcaaggattacccttccaacgaagaccttcacgaaaggctggaggttttcaaggccctcacagacaatgggagacacatcacctacttggaggaagagctggctgactttgtcctgcagtggatggatgttggcttgtcctcggaattccttctggtgctggtgaacttggtcaaattcaatagctgttacctcgacgagtacatcgcaaggatggttcagatgatctgtctgctgtgcgtccggaccgcgtcctctgtggacatagaggtctccctgcaggtgctggacgccgtggtctgctacaactgcctgccggctgagagcctcccgctgttcatcgttaccctctgtcgcaccatcaacgtcaaggagctctgcgagccttgctggaagctgatgcggaacctccttggcacccacctgggccacagcgccatctacaacatgtgccacctcatggaggacagagcctacatggaggacgcgcccctgctgagaggagccgtgttttttgtgggcatggctctctggggagcccaccggctctattctctcaggaactcgccgacatctgtgttgccatcattttaccaggccatggcatgtccgaacgaggtggtgtcctatgagatcgtcctgtccatcaccaggctcatcaagaagtataggaaggagctccaggtggtggcgtgggacattctgctgaacatcatcgaacggctccttcagcagctccagaccttggacagcccggagctcaggaccatcgtccatgacctgttgaccacggtggaggagctgtgtgaccagaacgagttccacgggtctcaggagagatactttgaactggtggagagatgtgcggaccagaggcctgagtcctccctcctgaacctgatctcctatagagcgcagtccatccacccggccaaggacggctggattcagaacctgcaggcgctgatggagagattcttcaggagcgagtcccgaggcgccgtgcgcatcaaggtgctggacgtgctgtcctttgtgctgctcatcaacaggcagttctatgaggaggagctgattaactcagtggtcatctcgcagctctcccacatccccgaggataaagaccaccaggtccgaaagctggccacccagttgctggtggacctggcagagggctgccacacacaccacttcaacagcctgctggacatcatcgagaaggtgatggcccgctccctctccccacccccggagctggaagaaagggatgtggccgcatactcggcctccttggaggatgtgaagacagccgtcctggggcttctggtcatccttcagaccaagctgtacaccctgcctgcaagccacgccacgcgtgtgtatgagatgctggtcagccacattcagctccactacaagcacagctacaccctgccaatcgcgagcagcatccggctgcaggcctttgacttcctgttgctgctgcgggccgactcactgcaccgcctgggcctgcccaacaaggatggagtcgtgcggttcagcccctactgcgtctgcgactacatggagccagagagaggctctgagaagaagaccagcggccccctttctcctcccacagggcctcctggcccggcgcctgcaggccccgccgtgcggctggggtccgtgccctactccctgctcttccgcgtcctgctgcagtgcttgaagcaggagtctgactggaaggtgctgaagctggttctgggcaggctgcctgagtccctgcgctataaagtgctcatctttacttccccttgcagtgtggaccagctgtgctctgctctctgctccatgctttcaggcccaaagacactggagcggctccgaggcgccccagaaggcttctccagaactgacttgcacctggccgtggttccagtgctgacagcattaatctcttaccataactacctggacaaaaccaaacagcgcgagatggtctactgcctggagcagggcctcatccaccgctgtgccagccagtgcgtcgtggccttgtccatctgcagcgtggagatgcctgacatcatcatcaaggcgctgcctgttctggtggtgaagctcacgcacatctcagccacagccagcatggccgtcccactgctggagttcctgtccactctggccaggctgccgcacctctacaggaactttgccgcggagcagtatgccagtgtgttcgccatctccctgccgtacaccaacccctccaagtttaatcagtacatcgtgtgtctggcccatcacgtcatagccatgtggttcatcaggtgccgcctgcccttccggaaggattttgtccctttcatcactaagggcctgcggtccaatgtcctcttgtcttttgatgacacccccgagaaggacagcttcagggcccggagtactagtctcaacgagagacccaagagtctgaggatagccagaccccccaaacaaggcttgaataactctccacccgtgaaagaattcaaggagagctctgcagccgaggccttccggtgccgcagcatcagtgtgtctgaacatgtggtccgcagcaggatacagacgtccctcaccagtgccagcttggggtctgcagatgagaactccgtggcccaggctgacgatagcctgaaaaacctccacctggagctcacggaaacctgtctggacatgatggctcgatacgtcttctccaacttcacggctgtcccgaagaggtctcctgtgggcgagttcctcctagcgggtggcaggaccaaaacctggctggttgggaacaagcttgtcactgtgacgacaagcgtgggaaccgggacccggtcgttactaggcctggactcgggggagctgcagtccggcccggagtcgagctccagccccggggtgcatgtgagacagaccaaggaggcgccggccaagctggagtcccaggctgggcagcaggtgtcccgtggggcccgggatcgggtccgttccatgtcggggggccatggtcttcgagttggcgccctggacgtgccggcctcccagttcctgggcagtgccacttctccaggaccacggactgcaccagccgcgaaacctgagaaggcctcagctggcacccgggttcctgtgcaggagaagacgaacctggcggcctatgtgcccctgctgacccagggctgggcggagatcctggtccggaggcccacagggaacaccagctggctgatgagcctggagaacccgctcagccctttctcctcggacatcaacaacatgcccctgcaggagctgtctaacgccctcatggcggctgagcgcttcaaggagcaccgggacacagccctgtacaagtcactgtcggtgccggcagccagcacggccaaaccccctcctctgcctcgctccaacacagtggcctctttctcctccctgtaccagtccagctgccaaggacagctgcacaggagcgtttcctgggcagactccgccgtggtcatggaggagggaagtccgggcgaggttcctgtgctggtggagcccccagggttggaggacgttgaggcagcgctaggcatggacaggcgcacggatgcctacagcaggtcgtcctcagtctccagccaggaggagaagtcgctccacgcggaggagctggttggcaggggcatccccatcgagcgagtcgtcgcntcggagggtggccggccctctgtggacctctccttccagccctcgcagcccctgagcaagtccagctcctctcccgagctgcagactctgcaggacatcctcggggaccctggggacaaggccgacgtgggccggctgagccctgaggttaaggcccggtcacagtcagggaccctggacggggaaagtgctgcctggtcggcctcgggcgaagacagtcggggccagcccgagggtcccttgccttccagctccccccgctcgcccagtggcctccggccccgaggttacaccatctccgactcggccccatcacgcaggggcaagagagtagagagggacgccttaaagagcagagccacagcctccaatgcagagaaagtgccaggcatcaaccccagtttcgtgttcctgcagctctaccattcccccttctttggcgacgagtcaaacaagccaatcctgctgcccaatgagtcacagtcctttgagcggtcggtgcagctcctcgaccagatcccatcatacgacacccacaagatcgccgtcctgtatgttggagaaggccagagcaacagcgagctcgccatcctgtccaatgagcatggctcctacaggtacacggagttcctgacgggcctgggccggctcatcgagctgaaggactgccagccggacaaggtgtacctgggaggcctggacgtgtgtggtgaggacggccagttcacctactgctggcacgatgacatcatgcaagccgtcttccacatcgccaccctgatgcccaccaaggacgtggacaagcaccgctgcgacaagaagcgccacctgggcaacgactttgtgtccattgtctacaatgactccggtgaggacttcaagcttggcaccatcaagggccagttcaactttgtccacgtgatcgtcaccccgctggactacgagtgcaacctggtgtccctgcagtgcaggaaagacatggagggccttgtggacaccagcgtggccaagatcgtgtctgaccgcaacctgcccttcgtggcccgccagatggccctgcacgcaaatatggcctcacaggtgcatcatagccgctccaaccccaccgatatctacccctccaagtggattgcccggctccgccacatcaagcggctccgccagcggatctgcgaggaagccgcctactccaaccccagcctacctctggtgcaccctccgtcccatagcaaagcccctgcacagactccagccgagcccacacctggctatgaggtgggccagcggaagcgcctcatctcctcggtggaggacttcaccgagtttgtgtga

SEQ ID NO: 15 - DNA, 5424 bp, Artificial
  nucleic acid sequence encoding an amino acid sequence of an exemplary engineered TSC2 polypeptide having a glutamic acid substitution at the serine residue at position S1364 of a human TSC2 polypeptide sequence
atggccaaaccaacaagcaaagattcaggcttgaaggagaagtttaagattctgttgggactgggaacaccgaggccaaatcccaggtctgcagagggtaaacagacggagtttatcatcaccgcggaaatactgagagaactgagcatggaatgtggcctcaacaatcgcatccggatgatagggcagatttgtgaagtcgcaaaaaccaagaaatttgaagagcacgcagtggaagcactctggaaggcggtcgcggatctgttgcagccggagcggccgctggaggcccggcacgcggtgctggctctgctgaaggccatcgtgcaggggcagggcgagcgtttgggggtcctcagagccctcttctttaaggtcatcaaggattacccttccaacgaagaccttcacgaaaggctggaggttttcaaggccctcacagacaatgggagacacatcacctacttggaggaagagctggctgactttgtcctgcagtggatggatgttggcttgtcctcggaattccttctggtgctggtgaacttggtcaaattcaatagctgttacctcgacgagtacatcgcaaggatggttcagatgatctgtctgctgtgcgtccggaccgcgtcctctgtggacatagaggtctccctgcaggtgctggacgccgtggtctgctacaactgcctgccggctgagagcctcccgctgttcatcgttaccctctgtcgcaccatcaacgtcaaggagctctgcgagccttgctggaagctgatgcggaacctccttggcacccacctgggccacagcgccatctacaacatgtgccacctcatggaggacagagcctacatggaggacgcgcccctgctgagaggagccgtgttttttgtgggcatggctctctggggagcccaccggctctattctctcaggaactcgccgacatctgtgttgccatcattttaccaggccatggcatgtccgaacgaggtggtgtcctatgagatcgtcctgtccatcaccaggctcatcaagaagtataggaaggagctccaggtggtggcgtgggacattctgctgaacatcatcgaacggctccttcagcagctccagaccttggacagcccggagctcaggaccatcgtccatgacctgttgaccacggtggaggagctgtgtgaccagaacgagttccacgggtctcaggagagatactttgaactggtggagagatgtgcggaccagaggcctgagtcctccctcctgaacctgatctcctatagagcgcagtccatccacccggccaaggacggctggattcagaacctgcaggcgctgatggagagattcttcaggagcgagtcccgaggcgccgtgcgcatcaaggtgctggacgtgctgtcctttgtgctgctcatcaacaggcagttctatgaggaggagctgattaactcagtggtcatctcgcagctctcccacatccccgaggataaagaccaccaggtccgaaagctggccacccagttgctggtggacctggcagagggctgccacacacaccacttcaacagcctgctggacatcatcgagaaggtgatggcccgctccctctccccacccccggagctggaagaaagggatgtggccgcatactcggcctccttggaggatgtgaagacagccgtcctggggcttctggtcatccttcagaccaagctgtacaccctgcctgcaagccacgccacgcgtgtgtatgagatgctggtcagccacattcagctccactacaagcacagctacaccctgccaatcgcgagcagcatccggctgcaggcctttgacttcctgttgctgctgcgggccgactcactgcaccgcctgggcctgcccaacaaggatggagtcgtgcggttcagcccctactgcgtctgcgactacatggagccagagagaggctctgagaagaagaccagcggccccctttctcctcccacagggcctcctggcccggcgcctgcaggccccgccgtgcggctggggtccgtgccctactccctgctcttccgcgtcctgctgcagtgcttgaagcaggagtctgactggaaggtgctgaagctggttctgggcaggctgcctgagtccctgcgctataaagtgctcatctttacttccccttgcagtgtggaccagctgtgctctgctctctgctccatgctttcaggcccaaagacactggagcggctccgaggcgccccagaaggcttctccagaactgacttgcacctggccgtggttccagtgctgacagcattaatctcttaccataactacctggacaaaaccaaacagcgcgagatggtctactgcctggagcagggcctcatccaccgctgtgccagccagtgcgtcgtggccttgtccatctgcagcgtggagatgcctgacatcatcatcaaggcgctgcctgttctggtggtgaagctcacgcacatctcagccacagccagcatggccgtcccactgctggagttcctgtccactctggccaggctgccgcacctctacaggaactttgccgcggagcagtatgccagtgtgttcgccatctccctgccgtacaccaacccctccaagtttaatcagtacatcgtgtgtctggcccatcacgtcatagccatgtggttcatcaggtgccgcctgcccttccggaaggattttgtccctttcatcactaagggcctgcggtccaatgtcctcttgtcttttgatgacacccccgagaaggacagcttcagggcccggagtactagtctcaacgagagacccaagagtctgaggatagccagaccccccaaacaaggcttgaataactctccacccgtgaaagaattcaaggagagctctgcagccgaggccttccggtgccgcagcatcagtgtgtctgaacatgtggtccgcagcaggatacagacgtccctcaccagtgccagcttggggtctgcagatgagaactccgtggcccaggctgacgatagcctgaaaaacctccacctggagctcacggaaacctgtctggacatgatggctcgatacgtcttctccaacttcacggctgtcccgaagaggtctcctgtgggcgagttcctcctagcgggtggcaggaccaaaacctggctggttgggaacaagcttgtcactgtgacgacaagcgtgggaaccgggacccggtcgttactaggcctggactcgggggagctgcagtccggcccggagtcgagctccagccccggggtgcatgtgagacagaccaaggaggcgccggccaagctggagtcccaggctgggcagcaggtgtcccgtggggcccgggatcgggtccgttccatgtcggggggccatggtcttcgagttggcgccctggacgtgccggcctcccagttcctgggcagtgccacttctccaggaccacggactgcaccagccgcgaaacctgagaaggcctcagctggcacccgggttcctgtgcaggagaagacgaacctggcggcctatgtgcccctgctgacccagggctgggcggagatcctggtccggaggcccacagggaacaccagctggctgatgagcctggagaacccgctcagccctttctcctcggacatcaacaacatgcccctgcaggagctgtctaacgccctcatggcggctgagcgcttcaaggagcaccgggacacagccctgtacaagtcactgtcggtgccggcagccagcacggccaaaccccctcctctgcctcgctccaacacagtggcctctttctcctccctgtaccagtccagctgccaaggacagctgcacaggagcgtttcctgggcagactccgccgtggtcatggaggagggaagtccgggcgaggttcctgtgctggtggagcccccagggttggaggacgttgaggcagcgctaggcatggacaggcgcacggatgcctacagcaggtcgtcctcagtctccagccaggaggagaagtcgctccacgcggaggagctggttggcaggggcatccccatcgagcgagtcgtcgartcggagggtggccggccctctgtggacctctccttccagccctcgcagcccctgagcaagtccagctcctctcccgagctgcagactctgcaggacatcctcggggaccctggggacaaggccgacgtgggccggctgagccctgaggttaaggcccggtcacagtcagggaccctggacggggaaagtgctgcctggtcggcctcgggcgaagacagtcggggccagcccgagggtcccttgccttccagctccccccgctcgcccagtggcctccggccccgaggttacaccatctccgactcggccccatcacgcaggggcaagagagtagagagggacgccttaaagagcagagccacagcctccaatgcagagaaagtgccaggcatcaaccccagtttcgtgttcctgcagctctaccattcccccttctttggcgacgagtcaaacaagccaatcctgctgcccaatgagtcacagtcctttgagcggtcggtgcagctcctcgaccagatcccatcatacgacacccacaagatcgccgtcctgtatgttggagaaggccagagcaacagcgagctcgccatcctgtccaatgagcatggctcctacaggtacacggagttcctgacgggcctgggccggctcatcgagctgaaggactgccagccggacaaggtgtacctgggaggcctggacgtgtgtggtgaggacggccagttcacctactgctggcacgatgacatcatgcaagccgtcttccacatcgccaccctgatgcccaccaaggacgtggacaagcaccgctgcgacaagaagcgccacctgggcaacgactttgtgtccattgtctacaatgactccggtgaggacttcaagcttggcaccatcaagggccagttcaactttgtccacgtgatcgtcaccccgctggactacgagtgcaacctggtgtccctgcagtgcaggaaagacatggagggccttgtggacaccagcgtggccaagatcgtgtctgaccgcaacctgcccttcgtggcccgccagatggccctgcacgcaaatatggcctcacaggtgcatcatagccgctccaaccccaccgatatctacccctccaagtggattgcccggctccgccacatcaagcggctccgccagcggatctgcgaggaagccgcctactccaaccccagcctacctctggtgcaccctccgtcccatagcaaagcccctgcacagactccagccgagcccacacctggctatgaggtgggccagcggaagcgcctcatctcctcggtggaggacttcaccgagtttgtgtga

SEQ ID NO: 16 - protein, 1814 aa, Artificial
  engineered TSC2 polypeptide having an alanine substitution at the serine residue at position S1365 of a mouse TSC2 polypeptide sequence
MAKPTSKDSGLKEKFKILLGLGTSRPNPRCAEGKQTEFIITSEILRELSGECGLNNRIRMIGQICDVAKTKKLEEHAVEALWKAVSDLLQPERPPEARHAVLTLLKAIVQGQGDRLGVLRALFFKVIKDYPSNEDLHERLEVFKALTDNGRHITYLEEELAEFVLQWMDVGLSSEFLLVLVNLVKFNSCYLDEYIASMVHMICLLCIRTVSSVDIEVSLQVLDAVVCYNCLPAESLPLFIITLCRTINVKELCEPCWKLMRNLLGTHLGHSAIYNMCRIMEDRSYMEDAPLLRGAVFFVGMALWGAHRLYSLKNSPTSVLPSFYEAMTCPNEVVSYEIVLSITRLIKKYRKELQAVTWDILLDIIERLLQQLQNLDSPELKTIVHDLLTTVEELCDQNEFHGSQERYYELVESYADQRPESSLLNLISYRAQSIHPAKDGWIQNLQLLMERFFRNECRSAVAIKVLDVLSFVLLIIRQFYEEELINSVVISQLSHIPEDKDHQVRKLATQLLVDLAEGCHTHHFNSLLDIIEKVMARSLSPPPELEERDLAVHSASLEDVKTAVLGLLVILQTKLYTLPASHATRVYESLISHIQLHYKHGYSLPIASSIRLQAFDFLLLLRADSLHRLGLPNKDGVVRFSPYCLCDCMELDRASEKKASGPLSPPTGPPSPVPMGPAVRLGYLPYSLLFRVLLQCLKQESDWKVLKLVLSRLPESLRYKVLIFTSPCSVDQLSSALCSMLSAPKTLERLRGTPEGFSRTDLHLAVVPVLTALISYHNYLDKTRQREMVYCLEQGLIYRCASQCVVALAICSVEMPDIIIKALPVLVVKLTHISATASMAIPLLEFLSTLARLPHLYRNFVPEQYASVFAISLPYTNPSKFNQYIVCLAHHVIAMWFIRCRLPFRKDFVPYITKGLRSNVLLSFDDTPEKDSFRARSTSLNERPKSLRIARAPKQGLNNSPPVKEFKESCAAEAFRCRSISVSEHVVRSRIQTSLTSASLGSADENSMAQADDNLKNLHLELTETCLDMMARYVFSNFTAVPKRSPVGEFLLAGGRTKTWLVGNKLVTVTTSVGTGTRSLLGLDSGDLQGGSDSSSDPSTHVRQTKEAPAKLESQAGQQVSRGARDRVRSMSGGHGLRVGVLDTSAPYSPGGSASLGPQTAVAAKPEKPPAGAQLPTAEKTNLAAYVPLLTQGWAEILVRRPTGNTSWLMSLENPLSPFSSDINNMPLQELSNALMAAERFKEHGHAPVQVIVSATGCTAKPPTLPRSNTVASFSSLYQPSCQGQLHRSVSWADSAMVLEEGSPGETQVPVEPPELEDFEAALGTDRHCQRPDTYSRSSSASSQEEKSHLEELAAGGIPIERAIASEGARPAVDLSFQPSQPLSKSSSSPELQTLQDILGDLGDKIDIGRLSPEAKVRSQSGILDGEAATWSATGEESRITVPPEGPLPSSSPRSPSGLRPRGYTISDSAPSRRGKRVERDNFKSRAAASSAEKVPGINPSFVFLQLYHSPFFGDESNKPILLPNESFERSVQLLDQIPSYDTHKIAVLYVGEGQSSSELAILSNEHGSYRYTEFLTGLGRLIELKDCQPDKVYLGGLDVCGEDGQFTYCWHDDIMQAVFHIATLMPTKDVDKHRCDKKRHLGNDFVSIIYNDSGEDFKLGTIKQGQFNFVHVIITPLDYKCNLLTLQCRKDGPACKCEWWRQPGEIVVWALPVVMELTVTILLCHLQMASQVHHSRSNPTDIYPSKWIARLRHIKRLRQRIREEVHYSNPSLPLMHPPAHTKAPAQAPEATPTYETGQRKRLISSVDDFTEFV

SEQ ID NO: 17 - protein, 1809 aa, Artificial
  engineered TSC2 polypeptide having an alanine substitution at the serine residue at position S1366 of a rat TSC2 polypeptide sequence
MAKPTSKDSGLKEKFKILLGLGTSRPNPRCAEGKQTEFIITAEILRELSGECGLNNRIRMIGQICDVAKTKKLEEHAVEALWKAVSDLLQPERPPEARHAVLALLKAIVQGQGDRLGVLRALFFKVIKDYPSNEDLHERLEVFKALTDNGRHITYLEEELAEFVLQWMDVGLSSEFLLVLVNLVKFNSCYLDEYIAPMVHMICLLCIRTVSSVDIEVSLQVLDAVVCYNCLPAESLPLFIITLCRTVNVKELCEPCWKLMRNLLGTHLGHSAIYNMCRIMENRSYMEDAPLLRGAVFFVGMALWGAHRLYSLKNSPTSVLPSFYEAMTCPNEVVSYEIVLSITRLIKKYRKELQAVTWDILLDIIERLLQQLQNLDSPELRTIVHDLLTTVEELCDQNEFHGSQERYYELVESYADQRPESSLLNLITYRAQSIHPAKDGWIQNLQLLMERFFRNECRSAVRIKVLDVLSFVLLINRQFYEEELINSVVISQLSHIPEDKDHQVRKLATQLLVDLAEGCHTHHFNSLLDIIEKVMARSLSPPLELEERDLAVYSASLEDVKTAVLGLLVILQTKLYTLPASHATRVYETLISHIQLHYKHGYSLPIASSIRLQAFDFLLLLRADSLHRLGLPNKDGVVRFSPYCLCDCAELDRASEKKASGPLSPPTGPPSPVPTGPAVRLGHLPYSLLFRVLLQCLKQETDWKVLKLVLSKLPESLRYKVLIFTSPCSVDQLSSALCSMLSAPKTLERLRGTPEGFSRTDLHLAVVPVLTALISYHNYLDKTRQREMVYCLEQGLIYRCASQCVVALAICSVEMPDIIIKALPVLVVKLTHISATASMAIPLLEFLSTLARLPHLYRNFAAEQYASVFAISLPYTNPSKFNQYIVCLAHHVIAMWFIRCRLPFRKDFVPYITKGLRSNVLLSFDDTPEKDKFRARSTSLNERPKSLRIARAPKQGLNNSPPVKEFKESCAAEAFRCRSISVSEHVVRSRIQTSLTSASLGSADENSMAQADDNLKNLHLELTETCLDMMARYVFSNFTAVPKRSPVGEFLLAGGRTKTWLVGNKLVTVTTSVGTGTRSLLGLDSGDLQGGSASSSDPGTHVRQTKEAPAKLESQAGQQVSRGARDRVRSMSGGHGLRVGVLDTSAPYTPGGPASLGAQAAPAARPEKPCAGAQLPAAEKANLAAYVPLLTQGWAEILVRRPTGNTSWLMSLENPLSPFSSDINNMPLQELSNALMAAERFKEHRDTALYKSLSVPAAGTAKPPTLPRSNTVASFSSLYQPSCQGQLHRSVSWADSAVVLEEGSPGEAHVPVEPPELEDFEAALGTDRHCQRPDAYSRSSSASSQEEKSHLEELAAGGIPIERAIASEGARPTVDLSFQPSQPLSKSSSSPELQTLQDILGDLGDKTDIGRLSPEAKVRSQSGILDGEAATWSAPGEESRITVPPEGPLPSSSPRSPSGLRPRGYTISDSAPSRRGKRVERDNFKSRTAASSAEKVPGINPSFVFLQLYHSPFCGDESNKPILLPNESFERSVQLLDQIPSYDTHKIAVLYVGEGQSSSELAILSNEHGSYRYTEFLTGLGRLIELKDCQPDKVYLGGLDVCGEDGQFTYCWHDDIMQAVFHIATLMPTKDVDKHRCDKKRHLGNDFVSIIYNDSGEDFKLGTIKGQFNFVHVIITPLDYKCNLLTLQCRKDMEGLVDTSVAKIVSDRNLSFVARQMALHANMASQVHHRRSNPTDIYPSKWIARLRHIKRLRQRIREEVHYSNPSLPLMHPPAHTKVPAQAPTEATPTYETGQRKRLISSVDDFTEFV

SEQ ID NO: 18 - protein, 1814 aa, Artificial
  engineered TSC2 polypeptide having a glutamic acid substitution at the serine residue at position S1365 of a mouse TSC2 polypeptide sequence
MAKPTSKDSGLKEKFKILLGLGTSRPNPRCAEGKQTEFIITSEILRELSGECGLNNRIRMIGQICDVAKTKKLEEHAVEALWKAVSDLLQPERPPEARHAVLTLLKAIVQGQGDRLGVLRALFFKVIKDYPSNEDLHERLEVFKALTDNGRHITYLEEELAEFVLQWMDVGLSSEFLLVLVNLVKFNSCYLDEYIASMVHMICLLCIRTVSSVDIEVSLQVLDAVVCYNCLPAESLPLFIITLCRTINVKELCEPCWKLMRNLLGTHLGHSAIYNMCRIMEDRSYMEDAPLLRGAVFFVGMALWGAHRLYSLKNSPTSVLPSFYEAMTCPNEVVSYEIVLSITRLIKKYRKELQAVTWDILLDIIERLLQQLQNLDSPELKTIVHDLLTTVEELCDQNEFHGSQERYYELVESYADQRPESSLLNLISYRAQSIHPAKDGWIQNLQLLMERFFRNECRSAVAIKVLDVLSFVLLIIRQFYEEELINSVVISQLSHIPEDKDHQVRKLATQLLVDLAEGCHTHHFNSLLDIIEKVMARSLSPPPELEERDLAVHSASLEDVKTAVLGLLVILQTKLYTLPASHATRVYESLISHIQLHYKHGYSLPIASSIRLQAFDFLLLLRADSLHRLGLPNKDGVVRFSPYCLCDCMELDRASEKKASGPLSPPTGPPSPVPMGPAVRLGYLPYSLLFRVLLQCLKQESDWKVLKLVLSRLPESLRYKVLIFTSPCSVDQLSSALCSMLSAPKTLERLRGTPEGFSRTDLHLAVVPVLTALISYHNYLDKTRQREMVYCLEQGLIYRCASQCVVALAICSVEMPDIIIKALPVLVVKLTHISATASMAIPLLEFLSTLARLPHLYRNFVPEQYASVFAISLPYTNPSKFNQYIVCLAHHVIAMWFIRCRLPFRKDFVPYITKGLRSNVLLSFDDTPEKDSFRARSTSLNERPKSLRIARAPKQGLNNSPPVKEFKESCAAEAFRCRSISVSEHVVRSRIQTSLTSASLGSADENSMAQADDNLKNLHLELTETCLDMMARYVFSNFTAVPKRSPVGEFLLAGGRTKTWLVGNKLVTVTTSVGTGTRSLLGLDSGDLQGGSDSSSDPSTHVRQTKEAPAKLESQAGQQVSRGARDRVRSMSGGHGLRVGVLDTSAPYSPGGSASLGPQTAVAAKPEKPPAGAQLPTAEKTNLAAYVPLLTQGWAEILVRRPTGNTSWLMSLENPLSPFSSDINNMPLQELSNALMAAERFKEHGHAPVQVIVSATGCTAKPPTLPRSNTVASFSSLYQPSCQGQLHRSVSWADSAMVLEEGSPGETQVPVEPPELEDFEAALGTDRHCQRPDTYSRSSSASSQEEKSHLEELAAGGIPIERAIESEGARPAVDLSFQPSQPLSKSSSSPELQTLQDILGDLGDKIDIGRLSPEAKVRSQSGILDGEAATWSATGEESRITVPPEGPLPSSSPRSPSGLRPRGYTISDSAPSRRGKRVERDNFKSRAAASSAEKVPGINPSFVFLQLYHSPFFGDESNKPILLPNESFERSVQLLDQIPSYDTHKIAVLYVGEGQSSSELAILSNEHGSYRYTEFLTGLGRLIELKDCQPDKVYLGGLDVCGEDGQFTYCWHDDIMQAVFHIATLMPTKDVDKHRCDKKRHLGNDFVSIIYNDSGEDFKLGTIKQGQFNFVHVIITPLDYKCNLLTLQCRKDGPACKCEWWRQPGEIVVWALPVVMELTVTILLCHLQMASQVHHSRSNPTDIYPSKWIARLRHIKRLRQRIREEVHYSNPSLPLMHPPAHTKAPAQAPEATPTYETGQRKRLISSVDDFTEFV

SEQ ID NO: 19 - protein, 1809 aa, Artificial
  engineered TSC2 polypeptide having a glutamic acid substitution at the serine residue at position S1366 of a rat TSC2 polypeptide sequence
MAKPTSKDSGLKEKFKILLGLGTSRPNPRCAEGKQTEFIITAEILRELSGECGLNNRIRMIGQICDVAKTKKLEEHAVEALWKAVSDLLQPERPPEARHAVLALLKAIVQGQGDRLGVLRALFFKVIKDYPSNEDLHERLEVFKALTDNGRHITYLEEELAEFVLQWMDVGLSSEFLLVLVNLVKFNSCYLDEYIAPMVHMICLLCIRTVSSVDIEVSLQVLDAVVCYNCLPAESLPLFIITLCRTVNVKELCEPCWKLMRNLLGTHLGHSAIYNMCRIMENRSYMEDAPLLRGAVFFVGMALWGAHRLYSLKNSPTSVLPSFYEAMTCPNEVVSYEIVLSITRLIKKYRKELQAVTWDILLDIIERLLQQLQNLDSPELRTIVHDLLTTVEELCDQNEFHGSQERYYELVESYADQRPESSLLNLITYRAQSIHPAKDGWIQNLQLLMERFFRNECRSAVRIKVLDVLSFVLLINRQFYEEELINSVVISQLSHIPEDKDHQVRKLATQLLVDLAEGCHTHHFNSLLDIIEKVMARSLSPPLELEERDLAVYSASLEDVKTAVLGLLVILQTKLYTLPASHATRVYETLISHIQLHYKHGYSLPIASSIRLQAFDFLLLLRADSLHRLGLPNKDGVVRFSPYCLCDCAELDRASEKKASGPLSPPTGPPSPVPTGPAVRLGHLPYSLLFRVLLQCLKQETDWKVLKLVLSKLPESLRYKVLIFTSPCSVDQLSSALCSMLSAPKTLERLRGTPEGFSRTDLHLAVVPVLTALISYHNYLDKTRQREMVYCLEQGLIYRCASQCVVALAICSVEMPDIIIKALPVLVVKLTHISATASMAIPLLEFLSTLARLPHLYRNFAAEQYASVFAISLPYTNPSKFNQYIVCLAHHVIAMWFIRCRLPFRKDFVPYITKGLRSNVLLSFDDTPEKDKFRARSTSLNERPKSLRIARAPKQGLNNSPPVKEFKESCAAEAFRCRSISVSEHVVRSRIQTSLTSASLGSADENSMAQADDNLKNLHLELTETCLDMMARYVFSNFTAVPKRSPVGEFLLAGGRTKTWLVGNKLVTVTTSVGTGTRSLLGLDSGDLQGGSASSSDPGTHVRQTKEAPAKLESQAGQQVSRGARDRVRSMSGGHGLRVGVLDTSAPYTPGGPASLGAQAAPAARPEKPCAGAQLPAAEKANLAAYVPLLTQGWAEILVRRPTGNTSWLMSLENPLSPFSSDINNMPLQELSNALMAAERFKEHRDTALYKSLSVPAAGTAKPPTLPRSNTVASFSSLYQPSCQGQLHRSVSWADSAVVLEEGSPGEAHVPVEPPELEDFEAALGTDRHCQRPDAYSRSSSASSQEEKSHLEELAAGGIPIERAIESEGARPTVDLSFQPSQPLSKSSSSPELQTLQDILGDLGDKTDIGRLSPEAKVRSQSGILDGEAATWSAPGEESRITVPPEGPLPSSSPRSPSGLRPRGYTISDSAPSRRGKRVERDNFKSRTAASSAEKVPGINPSFVFLQLYHSPFCGDESNKPILLPNESFERSVQLLDQIPSYDTHKIAVLYVGEGQSSSELAILSNEHGSYRYTEFLTGLGRLIELKDCQPDKVYLGGLDVCGEDGQFTYCWHDDIMQAVFHIATLMPTKDVDKHRCDKKRHLGNDFVSIIYNDSGEDFKLGTIKGQFNFVHVIITPLDYKCNLLTLQCRKDMEGLVDTSVAKIVSDRNLSFVARQMALHANMASQVHHRRSNPTDIYPSKWIARLRHIKRLRQRIREEVHYSNPSLPLMHPPAHTKVPAQAPTEATPTYETGQRKRLISSVDDFTEFV

SEQ ID NO: 20 - protein, 1807 aa, Artificial
  engineered TSC2 polypeptide having an alanine substitution at the serine residue at position S1364 and having an alanine substitution at the serine residue at position S1365 of a human TSC2 polypeptide sequence
MAKPTSKDSGLKEKFKILLGLGTPRPNPRSAEGKQTEFIITAEILRELSMECGLNNRIRMIGQICEVAKTKKFEEHAVEALWKAVADLLQPERPLEARHAVLALLKAIVQGQGERLGVLRALFFKVIKDYPSNEDLHERLEVFKALTDNGRHITYLEEELADFVLQWMDVGLSSEFLLVLVNLVKFNSCYLDEYIARMVQMICLLCVRTASSVDIEVSLQVLDAVVCYNCLPAESLPLFIVTLCRTINVKELCEPCWKLMRNLLGTHLGHSAIYNMCHLMEDRAYMEDAPLLRGAVFFVGMALWGAHRLYSLRNSPTSVLPSFYQAMACPNEVVSYEIVLSITRLIKKYRKELQVVAWDILLNIIERLLQQLQTLDSPELRTIVHDLLTTVEELCDQNEFHGSQERYFELVERCADQRPESSLLNLISYRAQSIHPAKDGWIQNLQALMERFFRSESRGAVRIKVLDVLSFVLLINRQFYEEELINSVVISQLSHIPEDKDHQVRKLATQLLVDLAEGCHTHHFNSLLDIIEKVMARSLSPPPELEERDVAAYSASLEDVKTAVLGLLVILQTKLYTLPASHATRVYEMLVSHIQLHYKHSYTLPIASSIRLQAFDFLLLLRADSLHRLGLPNKDGVVRFSPYCVCDYMEPERGSEKKTSGPLSPPTGPPGPAPAGPAVRLGSVPYSLLFRVLLQCLKQESDWKVLKLVLGRLPESLRYKVLIFTSPCSVDQLCSALCSMLSGPKTLERLRGAPEGFSRTDLHLAVVPVLTALISYHNYLDKTKQREMVYCLEQGLIHRCASQCVVALSICSVEMPDIIIKALPVLVVKLTHISATASMAVPLLEFLSTLARLPHLYRNFAAEQYASVFAISLPYTNPSKFNQYIVCLAHHVIAMWFIRCRLPFRKDFVPFITKGLRSNVLLSFDDTPEKDSFRARSTSLNERPKSLRIARPPKQGLNNSPPVKEFKESSAAEAFRCRSISVSEHVVRSRIQTSLTSASLGSADENSVAQADDSLKNLHLELTETCLDMMARYVFSNFTAVPKRSPVGEFLLAGGRTKTWLVGNKLVTVTTSVGTGTRSLLGLDSGELQSGPESSSSPGVHVRQTKEAPAKLESQAGQQVSRGARDRVRSMSGGHGLRVGALDVPASQFLGSATSPGPRTAPAAKPEKASAGTRVPVQEKTNLAAYVPLLTQGWAEILVRRPTGNTSWLMSLENPLSPFSSDINNMPLQELSNALMAAERFKEHRDTALYKSLSVPAASTAKPPPLPRSNTVASFSSLYQSSCQGQLHRSVSWADSAVVMEEGSPGEVPVLVEPPGLEDVEAALGMDRRTDAYSRSSSVSSQEEKSLHAEELVGRGIPIERVVAAEGGRPSVDLSFQPSQPLSKSSSSPELQTLQDILGDPGDKADVGRLSPEVKARSQSGTLDGESAAWSASGEDSRGQPEGPLPSSSPRSPSGLRPRGYTISDSAPSRRGKRVERDALKSRATASNAEKVPGINPSFVFLQLYHSPFFGDESNKPILLPNESQSFERSVQLLDQIPSYDTHKIAVLYVGEGQSNSELAILSNEHGSYRYTEFLTGLGRLIELKDCQPDKVYLGGLDVCGEDGQFTYCWHDDIMQAVFHIATLMPTKDVDKHRCDKKRHLGNDFVSIVYNDSGEDFKLGTIKGQFNFVHVIVTPLDYECNLVSLQCRKDMEGLVDTSVAKIVSDRNLPFVARQMALHANMASQVHHSRSNPTDIYPSKWIARLRHIKRLRQRICEEAAYSNPSLPLVHPPSHSKAPAQTPAEPTPGYEVGQRKRLISSVEDFTEFV

SEQ ID NO: 21 - protein, 1807 aa, Artificial
  engineered TSC2 polypeptide having a glutamic acid substitution at the serine residue at position S1364 and having a glutamic acid substitution at the serine residue at position S1365 of a human TSC2 polypeptide sequence
MAKPTSKDSGLKEKFKILLGLGTPRPNPRSAEGKQTEFIITAEILRELSMECGLNNRIRMIGQICEVAKTKKFEEHAVEALWKAVADLLQPERPLEARHAVLALLKAIVQGQGERLGVLRALFFKVIKDYPSNEDLHERLEVFKALTDNGRHITYLEEELADFVLQWMDVGLSSEFLLVLVNLVKFNSCYLDEYIARMVQMICLLCVRTASSVDIEVSLQVLDAVVCYNCLPAESLPLFIVTLCRTINVKELCEPCWKLMRNLLGTHLGHSAIYNMCHLMEDRAYMEDAPLLRGAVFFVGMALWGAHRLYSLRNSPTSVLPSFYQAMACPNEVVSYEIVLSITRLIKKYRKELQVVAWDILLNIIERLLQQLQTLDSPELRTIVHDLLTTVEELCDQNEFHGSQERYFELVERCADQRPESSLLNLISYRAQSIHPAKDGWIQNLQALMERFFRSESRGAVRIKVLDVLSFVLLINRQFYEEELINSVVISQLSHIPEDKDHQVRKLATQLLVDLAEGCHTHHFNSLLDIIEKVMARSLSPPPELEERDVAAYSASLEDVKTAVLGLLVILQTKLYTLPASHATRVYEMLVSHIQLHYKHSYTLPIASSIRLQAFDFLLLLRADSLHRLGLPNKDGVVRFSPYCVCDYMEPERGSEKKTSGPLSPPTGPPGPAPAGPAVRLGSVPYSLLFRVLLQCLKQESDWKVLKLVLGRLPESLRYKVLIFTSPCSVDQLCSALCSMLSGPKTLERLRGAPEGFSRTDLHLAVVPVLTALISYHNYLDKTKQREMVYCLEQGLIHRCASQCVVALSICSVEMPDIIIKALPVLVVKLTHISATASMAVPLLEFLSTLARLPHLYRNFAAEQYASVFAISLPYTNPSKFNQYIVCLAHHVIAMWFIRCRLPFRKDFVPFITKGLRSNVLLSFDDTPEKDSFRARSTSLNERPKSLRIARPPKQGLNNSPPVKEFKESSAAEAFRCRSISVSEHVVRSRIQTSLTSASLGSADENSVAQADDSLKNLHLELTETCLDMMARYVFSNFTAVPKRSPVGEFLLAGGRTKTWLVGNKLVTVTTSVGTGTRSLLGLDSGELQSGPESSSSPGVHVRQTKEAPAKLESQAGQQVSRGARDRVRSMSGGHGLRVGALDVPASQFLGSATSPGPRTAPAAKPEKASAGTRVPVQEKTNLAAYVPLLTQGWAEILVRRPTGNTSWLMSLENPLSPFSSDINNMPLQELSNALMAAERFKEHRDTALYKSLSVPAASTAKPPPLPRSNTVASFSSLYQSSCQGQLHRSVSWADSAVVMEEGSPGEVPVLVEPPGLEDVEAALGMDRRTDAYSRSSSVSSQEEKSLHAEELVGRGIPIERVVEEEGGRPSVDLSFQPSQPLSKSSSSPELQTLQDILGDPGDKADVGRLSPEVKARSQSGTLDGESAAWSASGEDSRGQPEGPLPSSSPRSPSGLRPRGYTISDSAPSRRGKRVERDALKSRATASNAEKVPGINPSFVFLQLYHSPFFGDESNKPILLPNESQSFERSVQLLDQIPSYDTHKIAVLYVGEGQSNSELAILSNEHGSYRYTEFLTGLGRLIELKDCQPDKVYLGGLDVCGEDGQFTYCWHDDIMQAVFHIATLMPTKDVDKHRCDKKRHLGNDFVSIVYNDSGEDFKLGTIKGQFNFVHVIVTPLDYECNLVSLQCRKDMEGLVDTSVAKIVSDRNLPFVARQMALHANMASQVHHSRSNPTDIYPSKWIARLRHIKRLRQRICEEAAYSNPSLPLVHPPSHSKAPAQTPAEPTPGYEVGQRKRLISSVEDFTEFV

SEQ ID NO: 22 - DNA, 5424 bp, Artificial
  nucleic acid sequence encoding an amino acid sequence of an exemplary engineered TSC2 polypeptide having an alanine substitution at the serine residue at position S1364 and having an alanine substitution at the serine residue at position S1365
  misc_feature (4092)..(4092): n is a, c, g, or t
  misc_feature (4095)..(4095): n is a, c, g, or t
atggccaaaccaacaagcaaagattcaggcttgaaggagaagtttaagattctgttgggactgggaacaccgaggccaaatcccaggtctgcagagggtaaacagacggagtttatcatcaccgcggaaatactgagagaactgagcatggaatgtggcctcaacaatcgcatccggatgatagggcagatttgtgaagtcgcaaaaaccaagaaatttgaagagcacgcagtggaagcactctggaaggcggtcgcggatctgttgcagccggagcggccgctggaggcccggcacgcggtgctggctctgctgaaggccatcgtgcaggggcagggcgagcgtttgggggtcctcagagccctcttctttaaggtcatcaaggattacccttccaacgaagaccttcacgaaaggctggaggttttcaaggccctcacagacaatgggagacacatcacctacttggaggaagagctggctgactttgtcctgcagtggatggatgttggcttgtcctcggaattccttctggtgctggtgaacttggtcaaattcaatagctgttacctcgacgagtacatcgcaaggatggttcagatgatctgtctgctgtgcgtccggaccgcgtcctctgtggacatagaggtctccctgcaggtgctggacgccgtggtctgctacaactgcctgccggctgagagcctcccgctgttcatcgttaccctctgtcgcaccatcaacgtcaaggagctctgcgagccttgctggaagctgatgcggaacctccttggcacccacctgggccacagcgccatctacaacatgtgccacctcatggaggacagagcctacatggaggacgcgcccctgctgagaggagccgtgttttttgtgggcatggctctctggggagcccaccggctctattctctcaggaactcgccgacatctgtgttgccatcattttaccaggccatggcatgtccgaacgaggtggtgtcctatgagatcgtcctgtccatcaccaggctcatcaagaagtataggaaggagctccaggtggtggcgtgggacattctgctgaacatcatcgaacggctccttcagcagctccagaccttggacagcccggagctcaggaccatcgtccatgacctgttgaccacggtggaggagctgtgtgaccagaacgagttccacgggtctcaggagagatactttgaactggtggagagatgtgcggaccagaggcctgagtcctccctcctgaacctgatctcctatagagcgcagtccatccacccggccaaggacggctggattcagaacctgcaggcgctgatggagagattcttcaggagcgagtcccgaggcgccgtgcgcatcaaggtgctggacgtgctgtcctttgtgctgctcatcaacaggcagttctatgaggaggagctgattaactcagtggtcatctcgcagctctcccacatccccgaggataaagaccaccaggtccgaaagctggccacccagttgctggtggacctggcagagggctgccacacacaccacttcaacagcctgctggacatcatcgagaaggtgatggcccgctccctctccccacccccggagctggaagaaagggatgtggccgcatactcggcctccttggaggatgtgaagacagccgtcctggggcttctggtcatccttcagaccaagctgtacaccctgcctgcaagccacgccacgcgtgtgtatgagatgctggtcagccacattcagctccactacaagcacagctacaccctgccaatcgcgagcagcatccggctgcaggcctttgacttcctgttgctgctgcgggccgactcactgcaccgcctgggcctgcccaacaaggatggagtcgtgcggttcagcccctactgcgtctgcgactacatggagccagagagaggctctgagaagaagaccagcggccccctttctcctcccacagggcctcctggcccggcgcctgcaggccccgccgtgcggctggggtccgtgccctactccctgctcttccgcgtcctgctgcagtgcttgaagcaggagtctgactggaaggtgctgaagctggttctgggcaggctgcctgagtccctgcgctataaagtgctcatctttacttccccttgcagtgtggaccagctgtgctctgctctctgctccatgctttcaggcccaaagacactggagcggctccgaggcgccccagaaggcttctccagaactgacttgcacctggccgtggttccagtgctgacagcattaatctcttaccataactacctggacaaaaccaaacagcgcgagatggtctactgcctggagcagggcctcatccaccgctgtgccagccagtgcgtcgtggccttgtccatctgcagcgtggagatgcctgacatcatcatcaaggcgctgcctgttctggtggtgaagctcacgcacatctcagccacagccagcatggccgtcccactgctggagttcctgtccactctggccaggctgccgcacctctacaggaactttgccgcggagcagtatgccagtgtgttcgccatctccctgccgtacaccaacccctccaagtttaatcagtacatcgtgtgtctggcccatcacgtcatagccatgtggttcatcaggtgccgcctgcccttccggaaggattttgtccctttcatcactaagggcctgcggtccaatgtcctcttgtcttttgatgacacccccgagaaggacagcttcagggcccggagtactagtctcaacgagagacccaagagtctgaggatagccagaccccccaaacaaggcttgaataactctccacccgtgaaagaattcaaggagagctctgcagccgaggccttccggtgccgcagcatcagtgtgtctgaacatgtggtccgcagcaggatacagacgtccctcaccagtgccagcttggggtctgcagatgagaactccgtggcccaggctgacgatagcctgaaaaacctccacctggagctcacggaaacctgtctggacatgatggctcgatacgtcttctccaacttcacggctgtcccgaagaggtctcctgtgggcgagttcctcctagcgggtggcaggaccaaaacctggctggttgggaacaagcttgtcactgtgacgacaagcgtgggaaccgggacccggtcgttactaggcctggactcgggggagctgcagtccggcccggagtcgagctccagccccggggtgcatgtgagacagaccaaggaggcgccggccaagctggagtcccaggctgggcagcaggtgtcccgtggggcccgggatcgggtccgttccatgtcggggggccatggtcttcgagttggcgccctggacgtgccggcctcccagttcctgggcagtgccacttctccaggaccacggactgcaccagccgcgaaacctgagaaggcctcagctggcacccgggttcctgtgcaggagaagacgaacctggcggcctatgtgcccctgctgacccagggctgggcggagatcctggtccggaggcccacagggaacaccagctggctgatgagcctggagaacccgctcagccctttctcctcggacatcaacaacatgcccctgcaggagctgtctaacgccctcatggcggctgagcgcttcaaggagcaccgggacacagccctgtacaagtcactgtcggtgccggcagccagcacggccaaaccccctcctctgcctcgctccaacacagtggcctctttctcctccctgtaccagtccagctgccaaggacagctgcacaggagcgtttcctgggcagactccgccgtggtcatggaggagggaagtccgggcgaggttcctgtgctggtggagcccccagggttggaggacgttgaggcagcgctaggcatggacaggcgcacggatgcctacagcaggtcgtcctcagtctccagccaggaggagaagtcgctccacgcggaggagctggttggcaggggcatccccatcgagcgagtcgtcgcngcngagggtggccggccctctgtggacctctccttccagccctcgcagcccctgagcaagtccagctcctctcccgagctgcagactctgcaggacatcctcggggaccctggggacaaggccgacgtgggccggctgagccctgaggttaaggcccggtcacagtcagggaccctggacggggaaagtgctgcctggtcggcctcgggcgaagacagtcggggccagcccgagggtcccttgccttccagctccccccgctcgcccagtggcctccggccccgaggttacaccatctccgactcggccccatcacgcaggggcaagagagtagagagggacgccttaaagagcagagccacagcctccaatgcagagaaagtgccaggcatcaaccccagtttcgtgttcctgcagctctaccattcccccttctttggcgacgagtcaaacaagccaatcctgctgcccaatgagtcacagtcctttgagcggtcggtgcagctcctcgaccagatcccatcatacgacacccacaagatcgccgtcctgtatgttggagaaggccagagcaacagcgagctcgccatcctgtccaatgagcatggctcctacaggtacacggagttcctgacgggcctgggccggctcatcgagctgaaggactgccagccggacaaggtgtacctgggaggcctggacgtgtgtggtgaggacggccagttcacctactgctggcacgatgacatcatgcaagccgtcttccacatcgccaccctgatgcccaccaaggacgtggacaagcaccgctgcgacaagaagcgccacctgggcaacgactttgtgtccattgtctacaatgactccggtgaggacttcaagcttggcaccatcaagggccagttcaactttgtccacgtgatcgtcaccccgctggactacgagtgcaacctggtgtccctgcagtgcaggaaagacatggagggccttgtggacaccagcgtggccaagatcgtgtctgaccgcaacctgcccttcgtggcccgccagatggccctgcacgcaaatatggcctcacaggtgcatcatagccgctccaaccccaccgatatctacccctccaagtggattgcccggctccgccacatcaagcggctccgccagcggatctgcgaggaagccgcctactccaaccccagcctacctctggtgcaccctccgtcccatagcaaagcccctgcacagactccagccgagcccacacctggctatgaggtgggccagcggaagcgcctcatctcctcggtggaggacttcaccgagtttgtgtga

SEQ ID NO: 23 - DNA, 5424 bp, Artificial
  nucleic acid sequence encoding an amino acid sequence of an exemplary engineered TSC2 polypeptide having a glutamic acid substitution at the serine residue at position S1364 and having a glutamic acid substitution at the serine residue at position
atggccaaaccaacaagcaaagattcaggcttgaaggagaagtttaagattctgttgggactgggaacaccgaggccaaatcccaggtctgcagagggtaaacagacggagtttatcatcaccgcggaaatactgagagaactgagcatggaatgtggcctcaacaatcgcatccggatgatagggcagatttgtgaagtcgcaaaaaccaagaaatttgaagagcacgcagtggaagcactctggaaggcggtcgcggatctgttgcagccggagcggccgctggaggcccggcacgcggtgctggctctgctgaaggccatcgtgcaggggcagggcgagcgtttgggggtcctcagagccctcttctttaaggtcatcaaggattacccttccaacgaagaccttcacgaaaggctggaggttttcaaggccctcacagacaatgggagacacatcacctacttggaggaagagctggctgactttgtcctgcagtggatggatgttggcttgtcctcggaattccttctggtgctggtgaacttggtcaaattcaatagctgttacctcgacgagtacatcgcaaggatggttcagatgatctgtctgctgtgcgtccggaccgcgtcctctgtggacatagaggtctccctgcaggtgctggacgccgtggtctgctacaactgcctgccggctgagagcctcccgctgttcatcgttaccctctgtcgcaccatcaacgtcaaggagctctgcgagccttgctggaagctgatgcggaacctccttggcacccacctgggccacagcgccatctacaacatgtgccacctcatggaggacagagcctacatggaggacgcgcccctgctgagaggagccgtgttttttgtgggcatggctctctggggagcccaccggctctattctctcaggaactcgccgacatctgtgttgccatcattttaccaggccatggcatgtccgaacgaggtggtgtcctatgagatcgtcctgtccatcaccaggctcatcaagaagtataggaaggagctccaggtggtggcgtgggacattctgctgaacatcatcgaacggctccttcagcagctccagaccttggacagcccggagctcaggaccatcgtccatgacctgttgaccacggtggaggagctgtgtgaccagaacgagttccacgggtctcaggagagatactttgaactggtggagagatgtgcggaccagaggcctgagtcctccctcctgaacctgatctcctatagagcgcagtccatccacccggccaaggacggctggattcagaacctgcaggcgctgatggagagattcttcaggagcgagtcccgaggcgccgtgcgcatcaaggtgctggacgtgctgtcctttgtgctgctcatcaacaggcagttctatgaggaggagctgattaactcagtggtcatctcgcagctctcccacatccccgaggataaagaccaccaggtccgaaagctggccacccagttgctggtggacctggcagagggctgccacacacaccacttcaacagcctgctggacatcatcgagaaggtgatggcccgctccctctccccacccccggagctggaagaaagggatgtggccgcatactcggcctccttggaggatgtgaagacagccgtcctggggcttctggtcatccttcagaccaagctgtacaccctgcctgcaagccacgccacgcgtgtgtatgagatgctggtcagccacattcagctccactacaagcacagctacaccctgccaatcgcgagcagcatccggctgcaggcctttgacttcctgttgctgctgcgggccgactcactgcaccgcctgggcctgcccaacaaggatggagtcgtgcggttcagcccctactgcgtctgcgactacatggagccagagagaggctctgagaagaagaccagcggccccctttctcctcccacagggcctcctggcccggcgcctgcaggccccgccgtgcggctggggtccgtgccctactccctgctcttccgcgtcctgctgcagtgcttgaagcaggagtctgactggaaggtgctgaagctggttctgggcaggctgcctgagtccctgcgctataaagtgctcatctttacttccccttgcagtgtggaccagctgtgctctgctctctgctccatgctttcaggcccaaagacactggagcggctccgaggcgccccagaaggcttctccagaactgacttgcacctggccgtggttccagtgctgacagcattaatctcttaccataactacctggacaaaaccaaacagcgcgagatggtctactgcctggagcagggcctcatccaccgctgtgccagccagtgcgtcgtggccttgtccatctgcagcgtggagatgcctgacatcatcatcaaggcgctgcctgttctggtggtgaagctcacgcacatctcagccacagccagcatggccgtcccactgctggagttcctgtccactctggccaggctgccgcacctctacaggaactttgccgcggagcagtatgccagtgtgttcgccatctccctgccgtacaccaacccctccaagtttaatcagtacatcgtgtgtctggcccatcacgtcatagccatgtggttcatcaggtgccgcctgcccttccggaaggattttgtccctttcatcactaagggcctgcggtccaatgtcctcttgtcttttgatgacacccccgagaaggacagcttcagggcccggagtactagtctcaacgagagacccaagagtctgaggatagccagaccccccaaacaaggcttgaataactctccacccgtgaaagaattcaaggagagctctgcagccgaggccttccggtgccgcagcatcagtgtgtctgaacatgtggtccgcagcaggatacagacgtccctcaccagtgccagcttggggtctgcagatgagaactccgtggcccaggctgacgatagcctgaaaaacctccacctggagctcacggaaacctgtctggacatgatggctcgatacgtcttctccaacttcacggctgtcccgaagaggtctcctgtgggcgagttcctcctagcgggtggcaggaccaaaacctggctggttgggaacaagcttgtcactgtgacgacaagcgtgggaaccgggacccggtcgttactaggcctggactcgggggagctgcagtccggcccggagtcgagctccagccccggggtgcatgtgagacagaccaaggaggcgccggccaagctggagtcccaggctgggcagcaggtgtcccgtggggcccgggatcgggtccgttccatgtcggggggccatggtcttcgagttggcgccctggacgtgccggcctcccagttcctgggcagtgccacttctccaggaccacggactgcaccagccgcgaaacctgagaaggcctcagctggcacccgggttcctgtgcaggagaagacgaacctggcggcctatgtgcccctgctgacccagggctgggcggagatcctggtccggaggcccacagggaacaccagctggctgatgagcctggagaacccgctcagccctttctcctcggacatcaacaacatgcccctgcaggagctgtctaacgccctcatggcggctgagcgcttcaaggagcaccgggacacagccctgtacaagtcactgtcggtgccggcagccagcacggccaaaccccctcctctgcctcgctccaacacagtggcctctttctcctccctgtaccagtccagctgccaaggacagctgcacaggagcgtttcctgggcagactccgccgtggtcatggaggagggaagtccgggcgaggttcctgtgctggtggagcccccagggttggaggacgttgaggcagcgctaggcatggacaggcgcacggatgcctacagcaggtcgtcctcagtctccagccaggaggagaagtcgctccacgcggaggagctggttggcaggggcatccccatcgagcgagtcgtcgargargagggtggccggccctctgtggacctctccttccagccctcgcagcccctgagcaagtccagctcctctcccgagctgcagactctgcaggacatcctcggggaccctggggacaaggccgacgtgggccggctgagccctgaggttaaggcccggtcacagtcagggaccctggacggggaaagtgctgcctggtcggcctcgggcgaagacagtcggggccagcccgagggtcccttgccttccagctccccccgctcgcccagtggcctccggccccgaggttacaccatctccgactcggccccatcacgcaggggcaagagagtagagagggacgccttaaagagcagagccacagcctccaatgcagagaaagtgccaggcatcaaccccagtttcgtgttcctgcagctctaccattcccccttctttggcgacgagtcaaacaagccaatcctgctgcccaatgagtcacagtcctttgagcggtcggtgcagctcctcgaccagatcccatcatacgacacccacaagatcgccgtcctgtatgttggagaaggccagagcaacagcgagctcgccatcctgtccaatgagcatggctcctacaggtacacggagttcctgacgggcctgggccggctcatcgagctgaaggactgccagccggacaaggtgtacctgggaggcctggacgtgtgtggtgaggacggccagttcacctactgctggcacgatgacatcatgcaagccgtcttccacatcgccaccctgatgcccaccaaggacgtggacaagcaccgctgcgacaagaagcgccacctgggcaacgactttgtgtccattgtctacaatgactccggtgaggacttcaagcttggcaccatcaagggccagttcaactttgtccacgtgatcgtcaccccgctggactacgagtgcaacctggtgtccctgcagtgcaggaaagacatggagggccttgtggacaccagcgtggccaagatcgtgtctgaccgcaacctgcccttcgtggcccgccagatggccctgcacgcaaatatggcctcacaggtgcatcatagccgctccaaccccaccgatatctacccctccaagtggattgcccggctccgccacatcaagcggctccgccagcggatctgcgaggaagccgcctactccaaccccagcctacctctggtgcaccctccgtcccatagcaaagcccctgcacagactccagccgagcccacacctggctatgaggtgggccagcggaagcgcctcatctcctcggtggaggacttcaccgagtttgtgtga

SEQ ID NO: 24 - protein, 1814 aa, Artificial
  engineered TSC2 polypeptide having an alanine substitution at the serine residue at position S1365 and having an alanine substitution at the serine residue at position S1366 of a mouse TSC2 polypeptide
MAKPTSKDSGLKEKFKILLGLGTSRPNPRCAEGKQTEFIITSEILRELSGECGLNNRIRMIGQICDVAKTKKLEEHAVEALWKAVSDLLQPERPPEARHAVLTLLKAIVQGQGDRLGVLRALFFKVIKDYPSNEDLHERLEVFKALTDNGRHITYLEEELAEFVLQWMDVGLSSEFLLVLVNLVKFNSCYLDEYIASMVHMICLLCIRTVSSVDIEVSLQVLDAVVCYNCLPAESLPLFIITLCRTINVKELCEPCWKLMRNLLGTHLGHSAIYNMCRIMEDRSYMEDAPLLRGAVFFVGMALWGAHRLYSLKNSPTSVLPSFYEAMTCPNEVVSYEIVLSITRLIKKYRKELQAVTWDILLDIIERLLQQLQNLDSPELKTIVHDLLTTVEELCDQNEFHGSQERYYELVESYADQRPESSLLNLISYRAQSIHPAKDGWIQNLQLLMERFFRNECRSAVAIKVLDVLSFVLLIIRQFYEEELINSVVISQLSHIPEDKDHQVRKLATQLLVDLAEGCHTHHFNSLLDIIEKVMARSLSPPPELEERDLAVHSASLEDVKTAVLGLLVILQTKLYTLPASHATRVYESLISHIQLHYKHGYSLPIASSIRLQAFDFLLLLRADSLHRLGLPNKDGVVRFSPYCLCDCMELDRASEKKASGPLSPPTGPPSPVPMGPAVRLGYLPYSLLFRVLLQCLKQESDWKVLKLVLSRLPESLRYKVLIFTSPCSVDQLSSALCSMLSAPKTLERLRGTPEGFSRTDLHLAVVPVLTALISYHNYLDKTRQREMVYCLEQGLIYRCASQCVVALAICSVEMPDIIIKALPVLVVKLTHISATASMAIPLLEFLSTLARLPHLYRNFVPEQYASVFAISLPYTNPSKFNQYIVCLAHHVIAMWFIRCRLPFRKDFVPYITKGLRSNVLLSFDDTPEKDSFRARSTSLNERPKSLRIARAPKQGLNNSPPVKEFKESCAAEAFRCRSISVSEHVVRSRIQTSLTSASLGSADENSMAQADDNLKNLHLELTETCLDMMARYVFSNFTAVPKRSPVGEFLLAGGRTKTWLVGNKLVTVTTSVGTGTRSLLGLDSGDLQGGSDSSSDPSTHVRQTKEAPAKLESQAGQQVSRGARDRVRSMSGGHGLRVGVLDTSAPYSPGGSASLGPQTAVAAKPEKPPAGAQLPTAEKTNLAAYVPLLTQGWAEILVRRPTGNTSWLMSLENPLSPFSSDINNMPLQELSNALMAAERFKEHGHAPVQVIVSATGCTAKPPTLPRSNTVASFSSLYQPSCQGQLHRSVSWADSAMVLEEGSPGETQVPVEPPELEDFEAALGTDRHCQRPDTYSRSSSASSQEEKSHLEELAAGGIPIERAIAAEGARPAVDLSFQPSQPLSKSSSSPELQTLQDILGDLGDKIDIGRLSPEAKVRSQSGILDGEAATWSATGEESRITVPPEGPLPSSSPRSPSGLRPRGYTISDSAPSRRGKRVERDNFKSRAAASSAEKVPGINPSFVFLQLYHSPFFGDESNKPILLPNESFERSVQLLDQIPSYDTHKIAVLYVGEGQSSSELAILSNEHGSYRYTEFLTGLGRLIELKDCQPDKVYLGGLDVCGEDGQFTYCWHDDIMQAVFHIATLMPTKDVDKHRCDKKRHLGNDFVSIIYNDSGEDFKLGTIKQGQFNFVHVIITPLDYKCNLLTLQCRKDGPACKCEWWRQPGEIVVWALPVVMELTVTILLCHLQMASQVHHSRSNPTDIYPSKWIARLRHIKRLRQRIREEVHYSNPSLPLMHPPAHTKAPAQAPEATPTYETGQRKRLISSVDDFTEFV

SEQ ID NO: 25 - protein, 1814 aa, Artificial
  engineered TSC2 polypeptide having an glutamic acid substitution at the serine residue at position S1365 and having an glutamic acid substitution at the serine residue at position S1366 of a mouse TSC2 polypeptide
MAKPTSKDSGLKEKFKILLGLGTSRPNPRCAEGKQTEFIITSEILRELSGECGLNNRIRMIGQICDVAKTKKLEEHAVEALWKAVSDLLQPERPPEARHAVLTLLKAIVQGQGDRLGVLRALFFKVIKDYPSNEDLHERLEVFKALTDNGRHITYLEEELAEFVLQWMDVGLSSEFLLVLVNLVKFNSCYLDEYIASMVHMICLLCIRTVSSVDIEVSLQVLDAVVCYNCLPAESLPLFIITLCRTINVKELCEPCWKLMRNLLGTHLGHSAIYNMCRIMEDRSYMEDAPLLRGAVFFVGMALWGAHRLYSLKNSPTSVLPSFYEAMTCPNEVVSYEIVLSITRLIKKYRKELQAVTWDILLDIIERLLQQLQNLDSPELKTIVHDLLTTVEELCDQNEFHGSQERYYELVESYADQRPESSLLNLISYRAQSIHPAKDGWIQNLQLLMERFFRNECRSAVAIKVLDVLSFVLLIIRQFYEEELINSVVISQLSHIPEDKDHQVRKLATQLLVDLAEGCHTHHFNSLLDIIEKVMARSLSPPPELEERDLAVHSASLEDVKTAVLGLLVILQTKLYTLPASHATRVYESLISHIQLHYKHGYSLPIASSIRLQAFDFLLLLRADSLHRLGLPNKDGVVRFSPYCLCDCMELDRASEKKASGPLSPPTGPPSPVPMGPAVRLGYLPYSLLFRVLLQCLKQESDWKVLKLVLSRLPESLRYKVLIFTSPCSVDQLSSALCSMLSAPKTLERLRGTPEGFSRTDLHLAVVPVLTALISYHNYLDKTRQREMVYCLEQGLIYRCASQCVVALAICSVEMPDIIIKALPVLVVKLTHISATASMAIPLLEFLSTLARLPHLYRNFVPEQYASVFAISLPYTNPSKFNQYIVCLAHHVIAMWFIRCRLPFRKDFVPYITKGLRSNVLLSFDDTPEKDSFRARSTSLNERPKSLRIARAPKQGLNNSPPVKEFKESCAAEAFRCRSISVSEHVVRSRIQTSLTSASLGSADENSMAQADDNLKNLHLELTETCLDMMARYVFSNFTAVPKRSPVGEFLLAGGRTKTWLVGNKLVTVTTSVGTGTRSLLGLDSGDLQGGSDSSSDPSTHVRQTKEAPAKLESQAGQQVSRGARDRVRSMSGGHGLRVGVLDTSAPYSPGGSASLGPQTAVAAKPEKPPAGAQLPTAEKTNLAAYVPLLTQGWAEILVRRPTGNTSWLMSLENPLSPFSSDINNMPLQELSNALMAAERFKEHGHAPVQVIVSATGCTAKPPTLPRSNTVASFSSLYQPSCQGQLHRSVSWADSAMVLEEGSPGETQVPVEPPELEDFEAALGTDRHCQRPDTYSRSSSASSQEEKSHLEELAAGGIPIERAIEEEGARPAVDLSFQPSQPLSKSSSSPELQTLQDILGDLGDKIDIGRLSPEAKVRSQSGILDGEAATWSATGEESRITVPPEGPLPSSSPRSPSGLRPRGYTISDSAPSRRGKRVERDNFKSRAAASSAEKVPGINPSFVFLQLYHSPFFGDESNKPILLPNESFERSVQLLDQIPSYDTHKIAVLYVGEGQSSSELAILSNEHGSYRYTEFLTGLGRLIELKDCQPDKVYLGGLDVCGEDGQFTYCWHDDIMQAVFHIATLMPTKDVDKHRCDKKRHLGNDFVSIIYNDSGEDFKLGTIKQGQFNFVHVIITPLDYKCNLLTLQCRKDGPACKCEWWRQPGEIVVWALPVVMELTVTILLCHLQMASQVHHSRSNPTDIYPSKWIARLRHIKRLRQRIREEVHYSNPSLPLMHPPAHTKAPAQAPEATPTYETGQRKRLISSVDDFTEFV

SEQ ID NO: 26 - protein, 1809 aa, Artificial
  engineered TSC2 polypeptide having an alanine substitution at the serine residue at position S1366 and having an alanine substitution at the serine residue at position S1367 of a rat TSC2 polypeptide
MAKPTSKDSGLKEKFKILLGLGTSRPNPRCAEGKQTEFIITAEILRELSGECGLNNRIRMIGQICDVAKTKKLEEHAVEALWKAVSDLLQPERPPEARHAVLALLKAIVQGQGDRLGVLRALFFKVIKDYPSNEDLHERLEVFKALTDNGRHITYLEEELAEFVLQWMDVGLSSEFLLVLVNLVKFNSCYLDEYIAPMVHMICLLCIRTVSSVDIEVSLQVLDAVVCYNCLPAESLPLFIITLCRTVNVKELCEPCWKLMRNLLGTHLGHSAIYNMCRIMENRSYMEDAPLLRGAVFFVGMALWGAHRLYSLKNSPTSVLPSFYEAMTCPNEVVSYEIVLSITRLIKKYRKELQAVTWDILLDIIERLLQQLQNLDSPELRTIVHDLLTTVEELCDQNEFHGSQERYYELVESYADQRPESSLLNLITYRAQSIHPAKDGWIQNLQLLMERFFRNECRSAVRIKVLDVLSFVLLINRQFYEEELINSVVISQLSHIPEDKDHQVRKLATQLLVDLAEGCHTHHFNSLLDIIEKVMARSLSPPLELEERDLAVYSASLEDVKTAVLGLLVILQTKLYTLPASHATRVYETLISHIQLHYKHGYSLPIASSIRLQAFDFLLLLRADSLHRLGLPNKDGVVRFSPYCLCDCAELDRASEKKASGPLSPPTGPPSPVPTGPAVRLGHLPYSLLFRVLLQCLKQETDWKVLKLVLSKLPESLRYKVLIFTSPCSVDQLSSALCSMLSAPKTLERLRGTPEGFSRTDLHLAVVPVLTALISYHNYLDKTRQREMVYCLEQGLIYRCASQCVVALAICSVEMPDIIIKALPVLVVKLTHISATASMAIPLLEFLSTLARLPHLYRNFAAEQYASVFAISLPYTNPSKFNQYIVCLAHHVIAMWFIRCRLPFRKDFVPYITKGLRSNVLLSFDDTPEKDKFRARSTSLNERPKSLRIARAPKQGLNNSPPVKEFKESCAAEAFRCRSISVSEHVVRSRIQTSLTSASLGSADENSMAQADDNLKNLHLELTETCLDMMARYVFSNFTAVPKRSPVGEFLLAGGRTKTWLVGNKLVTVTTSVGTGTRSLLGLDSGDLQGGSASSSDPGTHVRQTKEAPAKLESQAGQQVSRGARDRVRSMSGGHGLRVGVLDTSAPYTPGGPASLGAQAAPAARPEKPCAGAQLPAAEKANLAAYVPLLTQGWAEILVRRPTGNTSWLMSLENPLSPFSSDINNMPLQELSNALMAAERFKEHRDTALYKSLSVPAAGTAKPPTLPRSNTVASFSSLYQPSCQGQLHRSVSWADSAVVLEEGSPGEAHVPVEPPELEDFEAALGTDRHCQRPDAYSRSSSASSQEEKSHLEELAAGGIPIERAIAAEGARPTVDLSFQPSQPLSKSSSSPELQTLQDILGDLGDKTDIGRLSPEAKVRSQSGILDGEAATWSAPGEESRITVPPEGPLPSSSPRSPSGLRPRGYTISDSAPSRRGKRVERDNFKSRTAASSAEKVPGINPSFVFLQLYHSPFCGDESNKPILLPNESFERSVQLLDQIPSYDTHKIAVLYVGEGQSSSELAILSNEHGSYRYTEFLTGLGRLIELKDCQPDKVYLGGLDVCGEDGQFTYCWHDDIMQAVFHIATLMPTKDVDKHRCDKKRHLGNDFVSIIYNDSGEDFKLGTIKGQFNFVHVIITPLDYKCNLLTLQCRKDMEGLVDTSVAKIVSDRNLSFVARQMALHANMASQVHHRRSNPTDIYPSKWIARLRHIKRLRQRIREEVHYSNPSLPLMHPPAHTKVPAQAPTEATPTYETGQRKRLISSVDDFTEFV

SEQ ID NO: 27 - protein, 1809 aa, Artificial
  engineered TSC2 polypeptide having an glutamic acid substitution at the serine residue at position S1366 and having an glutamic acid substitution at the serine residue at position S1367 of a rat TSC2 polypeptide
MAKPTSKDSGLKEKFKILLGLGTSRPNPRCAEGKQTEFIITAEILRELSGECGLNNRIRMIGQICDVAKTKKLEEHAVEALWKAVSDLLQPERPPEARHAVLALLKAIVQGQGDRLGVLRALFFKVIKDYPSNEDLHERLEVFKALTDNGRHITYLEEELAEFVLQWMDVGLSSEFLLVLVNLVKFNSCYLDEYIAPMVHMICLLCIRTVSSVDIEVSLQVLDAVVCYNCLPAESLPLFIITLCRTVNVKELCEPCWKLMRNLLGTHLGHSAIYNMCRIMENRSYMEDAPLLRGAVFFVGMALWGAHRLYSLKNSPTSVLPSFYEAMTCPNEVVSYEIVLSITRLIKKYRKELQAVTWDILLDIIERLLQQLQNLDSPELRTIVHDLLTTVEELCDQNEFHGSQERYYELVESYADQRPESSLLNLITYRAQSIHPAKDGWIQNLQLLMERFFRNECRSAVRIKVLDVLSFVLLINRQFYEEELINSVVISQLSHIPEDKDHQVRKLATQLLVDLAEGCHTHHFNSLLDIIEKVMARSLSPPLELEERDLAVYSASLEDVKTAVLGLLVILQTKLYTLPASHATRVYETLISHIQLHYKHGYSLPIASSIRLQAFDFLLLLRADSLHRLGLPNKDGVVRFSPYCLCDCAELDRASEKKASGPLSPPTGPPSPVPTGPAVRLGHLPYSLLFRVLLQCLKQETDWKVLKLVLSKLPESLRYKVLIFTSPCSVDQLSSALCSMLSAPKTLERLRGTPEGFSRTDLHLAVVPVLTALISYHNYLDKTRQREMVYCLEQGLIYRCASQCVVALAICSVEMPDIIIKALPVLVVKLTHISATASMAIPLLEFLSTLARLPHLYRNFAAEQYASVFAISLPYTNPSKFNQYIVCLAHHVIAMWFIRCRLPFRKDFVPYITKGLRSNVLLSFDDTPEKDKFRARSTSLNERPKSLRIARAPKQGLNNSPPVKEFKESCAAEAFRCRSISVSEHVVRSRIQTSLTSASLGSADENSMAQADDNLKNLHLELTETCLDMMARYVFSNFTAVPKRSPVGEFLLAGGRTKTWLVGNKLVTVTTSVGTGTRSLLGLDSGDLQGGSASSSDPGTHVRQTKEAPAKLESQAGQQVSRGARDRVRSMSGGHGLRVGVLDTSAPYTPGGPASLGAQAAPAARPEKPCAGAQLPAAEKANLAAYVPLLTQGWAEILVRRPTGNTSWLMSLENPLSPFSSDINNMPLQELSNALMAAERFKEHRDTALYKSLSVPAAGTAKPPTLPRSNTVASFSSLYQPSCQGQLHRSVSWADSAVVLEEGSPGEAHVPVEPPELEDFEAALGTDRHCQRPDAYSRSSSASSQEEKSHLEELAAGGIPIERAIEEEGARPTVDLSFQPSQPLSKSSSSPELQTLQDILGDLGDKTDIGRLSPEAKVRSQSGILDGEAATWSAPGEESRITVPPEGPLPSSSPRSPSGLRPRGYTISDSAPSRRGKRVERDNFKSRTAASSAEKVPGINPSFVFLQLYHSPFCGDESNKPILLPNESFERSVQLLDQIPSYDTHKIAVLYVGEGQSSSELAILSNEHGSYRYTEFLTGLGRLIELKDCQPDKVYLGGLDVCGEDGQFTYCWHDDIMQAVFHIATLMPTKDVDKHRCDKKRHLGNDFVSIIYNDSGEDFKLGTIKGQFNFVHVIITPLDYKCNLLTLQCRKDMEGLVDTSVAKIVSDRNLSFVARQMALHANMASQVHHRRSNPTDIYPSKWIARLRHIKRLRQRIREEVHYSNPSLPLMHPPAHTKVPAQAPTEATPTYETGQRKRLISSVDDFTEFV